European Patent Application EP 4 745 242 A1, published May 20, 2026. Title: 核酸载体、核酸药及其制备方法和应用. Applicant: 百药智达（北京）纳米生物技术有限公司. Application CN. The sequence listing filed with the application follows.

SEQUENCE LISTING (535 sequences)

SEQ ID NO: 1 - DNA, 12 bp, synthetic construct
  source 1..12: mol_type = other DNA
acgagcgttccg

SEQ ID NO: 2 - DNA, 10 bp, synthetic construct
  source 1..10: mol_type = other DNA
cggttcgccg

SEQ ID NO: 3 - DNA, 13 bp, synthetic construct
  source 1..13: mol_type = other DNA
cggccatagccgt

SEQ ID NO: 4 - RNA, 12 nt, synthetic construct
  source 1..12: mol_type = other RNA
acgagcgttccg

SEQ ID NO: 5 - RNA, 10 nt, synthetic construct
  source 1..10: mol_type = other RNA
cggttcgccg

SEQ ID NO: 6 - RNA, 13 nt, synthetic construct
  source 1..13: mol_type = other RNA
cggccatagccgt

SEQ ID NO: 7 - DNA, 14 bp, synthetic construct
  source 1..14: mol_type = other DNA
tgtagcacggtggc

SEQ ID NO: 8 - DNA, 14 bp, synthetic construct
  source 1..14: mol_type = other DNA
gccaccgtgctaca

SEQ ID NO: 9 - DNA, 14 bp, synthetic construct
  source 1..14: mol_type = other DNA
tcggcgcggccgtg

SEQ ID NO: 10 - DNA, 14 bp, synthetic construct
  source 1..14: mol_type = other DNA
cacggccgcgccga

SEQ ID NO: 11 - DNA, 14 bp, synthetic construct
  source 1..14: mol_type = other DNA
tgctgctgctgctg

SEQ ID NO: 12 - DNA, 14 bp, synthetic construct
  source 1..14: mol_type = other DNA
cagcagcagcagca

SEQ ID NO: 13 - DNA, 14 bp, synthetic construct
  source 1..14: mol_type = other DNA
cgcggctcgcggct

SEQ ID NO: 14 - DNA, 14 bp, synthetic construct
  source 1..14: mol_type = other DNA
agccgcgagccgcg

SEQ ID NO: 15 - DNA, 40 bp, synthetic construct
  source 1..40: mol_type = other DNA
gacgcccacgagcgttccgggagaggtgtagcacggtggc

SEQ ID NO: 16 - DNA, 37 bp, synthetic construct
  source 1..37: mol_type = other DNA
cctctcccggttcgccgcgagcctcggcgcggccgtg

SEQ ID NO: 17 - DNA, 40 bp, synthetic construct
  source 1..40: mol_type = other DNA
ggctcgcggccatagccgtgggcgtctgctgctgctgctg

SEQ ID NO: 18 - DNA, 31 bp, synthetic construct
  source 1..31: mol_type = other DNA
gcgacgcccacgagcgttccgggagaggagc

SEQ ID NO: 19 - DNA, 29 bp, synthetic construct
  source 1..29: mol_type = other DNA
gctcctctcccggttcgccgcgagccgcg

SEQ ID NO: 20 - DNA, 45 bp, synthetic construct
  source 1..45: mol_type = other DNA
cagcagcagcagcacgcggctcgcggccatagccgtgggcgtcgc

SEQ ID NO: 21 - DNA, 30 bp, synthetic construct
  source 1..30: mol_type = other DNA
gcgacgcccacgagcgttccgggagaggag

SEQ ID NO: 22 - DNA, 28 bp, synthetic construct
  source 1..28: mol_type = other DNA
ctcctctcccggttcgccgcgagccgcg

SEQ ID NO: 23 - DNA, 31 bp, synthetic construct
  source 1..31: mol_type = other DNA
cgcggcacgcggccatagccgtgggcgtcgc

SEQ ID NO: 24 - DNA, 32 bp, synthetic construct
  source 1..32: mol_type = other DNA
gcgacgcccacgagcgttccgggagaggagct

SEQ ID NO: 25 - DNA, 30 bp, synthetic construct
  source 1..30: mol_type = other DNA
gctcctctcccggttcgccgcgagccgcgt

SEQ ID NO: 26 - DNA, 32 bp, synthetic construct
  source 1..32: mol_type = other DNA
cgcggctcgcggccatagccgtgggcgtcgct

SEQ ID NO: 27 - DNA, 32 bp, synthetic construct
  source 1..32: mol_type = other DNA
cgcggcacgcggccatagccgtgggcgtcgct

SEQ ID NO: 28 - DNA, 26 bp, synthetic construct
  source 1..26: mol_type = other DNA
gacgcccacgagcgttccgggagagg

SEQ ID NO: 29 - DNA, 23 bp, synthetic construct
  source 1..23: mol_type = other DNA
cctctcccggttcgccgcgagcc

SEQ ID NO: 30 - DNA, 26 bp, synthetic construct
  source 1..26: mol_type = other DNA
ggctcgcggccatagccgtgggcgtc

SEQ ID NO: 31 - DNA, 31 bp, synthetic construct
  source 1..31: mol_type = other DNA
cgcggctcgcggccatagccgtgggcgtcgc

SEQ ID NO: 32 - DNA, 30 bp, synthetic construct
  source 1..30: mol_type = other DNA
cgacgcccacgagcgttccgggagaggagc

SEQ ID NO: 33 - DNA, 26 bp, synthetic construct
  source 1..26: mol_type = other DNA
gcggcgcccacgagcgttccgggagc

SEQ ID NO: 34 - DNA, 24 bp, synthetic construct
  source 1..24: mol_type = other DNA
gctcccggttcgccgccagccgcc

SEQ ID NO: 35 - DNA, 31 bp, synthetic construct
  source 1..31: mol_type = other DNA
ggcggcaggcggccatagccgtgggcgccgc

SEQ ID NO: 36 - DNA, 30 bp, synthetic construct
  source 1..30: mol_type = other DNA
gcggcgcccacgagcgttccgggagaggcc

SEQ ID NO: 37 - DNA, 30 bp, synthetic construct; identical to SEQ ID NO: 36
  source 1..30: mol_type = other DNA

SEQ ID NO: 38 - DNA, 31 bp, synthetic construct
  source 1..31: mol_type = other DNA
ggcggctggcggccatagccgtgggcgccgc

SEQ ID NO: 39 - DNA, 31 bp, synthetic construct
  source 1..31: mol_type = other DNA
gcggcgcccacgagcgttccgggagaggcct

SEQ ID NO: 40 - DNA, 29 bp, synthetic construct
  source 1..29: mol_type = other DNA
ggcctctcccggttcgccgccagccgcct

SEQ ID NO: 41 - DNA, 32 bp, synthetic construct
  source 1..32: mol_type = other DNA
ggcggctggcggccatagccgtgggcgccgct

SEQ ID NO: 42 - RNA, 30 nt, synthetic construct
  source 1..30: mol_type = other RNA
gcggcgcccacgagcgttccgggagaggcc

SEQ ID NO: 43 - RNA, 28 nt, synthetic construct
  source 1..28: mol_type = other RNA
ggcctctcccggttcgccgccagccgcc

SEQ ID NO: 44 - RNA, 31 nt, synthetic construct
  source 1..31: mol_type = other RNA
ggcggctggcggccatagccgtgggcgccgc

SEQ ID NO: 45 - DNA, 29 bp, synthetic construct
  source 1..29: mol_type = other DNA
cgacgcccacgagcgttccgggagaggag

SEQ ID NO: 46 - DNA, 28 bp, synthetic construct
  source 1..28: mol_type = other DNA
ctcctctcccggttcgccgccagccgcc

SEQ ID NO: 47 - DNA, 30 bp, synthetic construct
  source 1..30: mol_type = other DNA
gcggcgcccacgagcgttccgggagaggag

SEQ ID NO: 48 - DNA, 22 bp, synthetic construct
  source 1..22: mol_type = other DNA
cgcccacgagcgttccgggaga

SEQ ID NO: 49 - DNA, 19 bp, synthetic construct
  source 1..19: mol_type = other DNA
tctcccggttcgccgcgag

SEQ ID NO: 50 - DNA, 22 bp, synthetic construct
  source 1..22: mol_type = other DNA
ctcgcggccatagccgtgggcg

SEQ ID NO: 51 - RNA, 23 nt, synthetic construct
  source 1..23: mol_type = other RNA
tcgcccacgagcgttccgggaga

SEQ ID NO: 52 - RNA, 19 nt, synthetic construct
  source 1..19: mol_type = other RNA
tctcccggttcgccgcgag

SEQ ID NO: 53 - RNA, 23 nt, synthetic construct
  source 1..23: mol_type = other RNA
tctcgcggccatagccgtgggcg

SEQ ID NO: 54 - DNA, 25 bp, synthetic construct
  source 1..25: mol_type = other DNA
gcgcccacgagcgttccgggagagc

SEQ ID NO: 55 - DNA, 30 bp, synthetic construct
  source 1..30: mol_type = other DNA
  misc_feature 4: note = RNA
  misc_feature 1..3: note = DNA
  misc_feature 5..30: note = DNA
ccctgctctcccggttcgccgccagccgcc

SEQ ID NO: 56 - DNA, 28 bp, synthetic construct
  source 1..28: mol_type = other DNA
ggcggcaggcggccatagccgtgggcgc

SEQ ID NO: 57 - DNA, 24 bp, synthetic construct
  source 1..24: mol_type = other DNA
tcgtcgttttgtcgttttgtcgtt

SEQ ID NO: 58 - RNA, 24 nt, synthetic construct
  source 1..24: mol_type = other RNA
tcgtcgttttgtcgttttgtcgtt

SEQ ID NO: 59 - DNA, 18 bp, synthetic construct
  source 1..18: mol_type = other DNA
tccatgacgttcctgacg

SEQ ID NO: 60 - DNA, 20 bp, synthetic construct
  source 1..20: mol_type = other DNA
gggggacgatcgtcgggggg

SEQ ID NO: 61 - DNA, 22 bp, synthetic construct
  source 1..22: mol_type = other DNA
tcgtcgttttcggcgcgcgccg

SEQ ID NO: 62 - DNA, 21 bp, synthetic construct
  source 1..21: mol_type = other DNA
tcgtcgtcgtcgtcgtcgtcg

SEQ ID NO: 63 - DNA, 24 bp, synthetic construct
  source 1..24: mol_type = other DNA
tcgtcgtcgtcgtcgtcgtcgtcg

SEQ ID NO: 64 - RNA, 21 nt, synthetic construct
  source 1..21: mol_type = other RNA
atttgcttccataatatcatt

SEQ ID NO: 65 - RNA, 21 nt, synthetic construct
  source 1..21: mol_type = other RNA
tgatattatggaagcaaattt

SEQ ID NO: 66 - RNA, 21 nt, synthetic construct
  source 1..21: mol_type = other RNA
ttaggtttggggttggatctt

SEQ ID NO: 67 - RNA, 21 nt, synthetic construct
  source 1..21: mol_type = other RNA
gatccaaccccaaacctaatt

SEQ ID NO: 68 - RNA, 21 nt, synthetic construct
  source 1..21: mol_type = other RNA
gcgtcgaagttgtaggatttt

SEQ ID NO: 69 - RNA, 21 nt, synthetic construct
  source 1..21: mol_type = other RNA
aatcctacaacttcgacgctt

SEQ ID NO: 70 - RNA, 21 nt, synthetic construct
  source 1..21: mol_type = other RNA
tgtttacattgttgaggtatt

SEQ ID NO: 71 - RNA, 21 nt, synthetic construct
  source 1..21: mol_type = other RNA
tacctcaacaatgtaaacttt

SEQ ID NO: 72 - DNA, 21 bp, synthetic construct
  misc_feature 20..21: note = dTdT
  source 1..21: mol_type = other DNA
  misc_feature 1..19: note = RNA
ggtgattacccagagatattt

SEQ ID NO: 73 - DNA, 21 bp, synthetic construct
  misc_feature 20..21: note = dTdT
  source 1..21: mol_type = other DNA
  misc_feature 1..19: note = RNA
atatctctgggtaatcacctt

SEQ ID NO: 74 - RNA, 21 nt, synthetic construct
  source 1..21: mol_type = other RNA
tggtgaaagaggtcattcctt

SEQ ID NO: 75 - RNA, 21 nt, synthetic construct
  source 1..21: mol_type = other RNA
ggaatgacctctttcaccatt

SEQ ID NO: 76 - RNA, 21 nt, synthetic construct
  source 1..21: mol_type = other RNA
  misc_feature 20..21: note = dTdT
ggaatgacctctttcaccatt

SEQ ID NO: 77 - DNA, 21 bp, synthetic construct
  misc_feature 20..21: note = dTdT
  source 1..21: mol_type = other DNA
  misc_feature 1..19: note = RNA
tggtgaaagaggtcattcctt

SEQ ID NO: 78 - RNA, 21 nt, synthetic construct
  source 1..21: mol_type = other RNA
ggtgattacccagagatattt

SEQ ID NO: 79 - RNA, 21 nt, synthetic construct
  source 1..21: mol_type = other RNA
atatctctgggtaatcacctt

SEQ ID NO: 80 - RNA, 21 nt, synthetic construct
  source 1..21: mol_type = other RNA
ggctggttatgtcctcatttt

SEQ ID NO: 81 - RNA, 21 nt, synthetic construct
  source 1..21: mol_type = other RNA
aatgaggacataaccagcctt

SEQ ID NO: 82 - RNA, 21 nt, synthetic construct
  source 1..21: mol_type = other RNA
ccttagcagtcttatctaatt

SEQ ID NO: 83 - RNA, 21 nt, synthetic construct
  source 1..21: mol_type = other RNA
ttagataagactgctaaggtt

SEQ ID NO: 84 - RNA, 23 nt, synthetic construct
  source 1..23: mol_type = other RNA
tgccttagcagtcttatctaatt

SEQ ID NO: 85 - RNA, 23 nt, synthetic construct
  source 1..23: mol_type = other RNA
ttagataagactgctaaggcatt

SEQ ID NO: 86 - RNA, 25 nt, synthetic construct
  source 1..25: mol_type = other RNA
tgccttagcagtcttatctaatttt

SEQ ID NO: 87 - RNA, 25 nt, synthetic construct
  source 1..25: mol_type = other RNA
aattagataagactgctaaggcatt

SEQ ID NO: 88 - RNA, 21 nt, synthetic construct
  source 1..21: mol_type = other RNA
ggacttctctcaattttcttt

SEQ ID NO: 89 - RNA, 21 nt, synthetic construct
  source 1..21: mol_type = other RNA
agaaaattgagagaagtcctt

SEQ ID NO: 90 - RNA, 21 nt, synthetic construct
  source 1..21: mol_type = other RNA
cgcagaacaccgtgttcgatt

SEQ ID NO: 91 - RNA, 21 nt, synthetic construct
  source 1..21: mol_type = other RNA
tcgaacacggtgttctgcgtt

SEQ ID NO: 92 - RNA, 21 nt, synthetic construct
  source 1..21: mol_type = other RNA
ggccaacaagatcaccatctt

SEQ ID NO: 93 - RNA, 21 nt, synthetic construct
  source 1..21: mol_type = other RNA
gatggtgatcttgttggcctt

SEQ ID NO: 94 - RNA, 21 nt, synthetic construct
  source 1..21: mol_type = other RNA
ccagcacactgagaatcaatt

SEQ ID NO: 95 - RNA, 21 nt, synthetic construct
  source 1..21: mol_type = other RNA
ttgattctcagtgtgctggtt

SEQ ID NO: 96 - DNA, 21 bp, synthetic construct
  misc_feature 20..21: note = dTdT
  source 1..21: mol_type = other DNA
  misc_feature 1..19: note = RNA
agacgtaagcagtgttgaatt

SEQ ID NO: 97 - DNA, 21 bp, synthetic construct
  misc_feature 20..21: note = dTdT
  source 1..21: mol_type = other DNA
  misc_feature 1..19: note = RNA
ttcaacactgcttacgtcttt

SEQ ID NO: 98 - DNA, 21 bp, synthetic construct
  misc_feature 20..21: note = dTdT
  source 1..21: mol_type = other DNA
  misc_feature 1..19: note = RNA
gaggaaggtatcaacaaattt

SEQ ID NO: 99 - DNA, 21 bp, synthetic construct
  misc_feature 20..21: note = dTdT
  source 1..21: mol_type = other DNA
  misc_feature 1..19: note = RNA
atttgttgataccttcctctt

SEQ ID NO: 100 - RNA, 23 nt, synthetic construct
  source 1..23: mol_type = other RNA
gcaggttccttatctgtcacatt

SEQ ID NO: 101 - RNA, 23 nt, synthetic construct
  source 1..23: mol_type = other RNA
tgtgacagataaggaacctgctt

SEQ ID NO: 102 - RNA, 23 nt, synthetic construct
  source 1..23: mol_type = other RNA
ggaattggaaggctgggaacctt

SEQ ID NO: 103 - RNA, 23 nt, synthetic construct
  source 1..23: mol_type = other RNA
ggttcccagccttccaattcctt

SEQ ID NO: 104 - DNA, 22 bp, synthetic construct
  misc_feature 21..22: note = dTdT
  source 1..22: mol_type = other DNA
  misc_feature 1..20: note = RNA
tgcaggttccttatctgtcatt

SEQ ID NO: 105 - DNA, 21 bp, synthetic construct
  misc_feature 20..21: note = dTdT
  source 1..21: mol_type = other DNA
  misc_feature 1..19: note = RNA
tgacagataaggaacctgctt

SEQ ID NO: 106 - RNA, 25 nt, synthetic construct
  source 1..25: mol_type = other RNA
ctgcaggttccttatctgtcacatt

SEQ ID NO: 107 - RNA, 25 nt, synthetic construct
  source 1..25: mol_type = other RNA
tgtgacagataaggaacctgcagtt

SEQ ID NO: 108 - RNA, 21 nt, synthetic construct
  source 1..21: mol_type = other RNA
gctgcacacggttcagaattt

SEQ ID NO: 109 - RNA, 21 nt, synthetic construct
  source 1..21: mol_type = other RNA
attctgaaccgtgtgcagctt

SEQ ID NO: 110 - RNA, 21 nt, synthetic construct
  source 1..21: mol_type = other RNA
caggatgagttacttgaaatt

SEQ ID NO: 111 - RNA, 21 nt, synthetic construct
  source 1..21: mol_type = other RNA
tttcaagtaactcatcctgtt

SEQ ID NO: 112 - DNA, 21 bp, synthetic construct
  misc_feature 20..21: note = dTdT
  source 1..21: mol_type = other DNA
  misc_feature 1..19: note = RNA
gtgctcaggactgatgaaatt

SEQ ID NO: 113 - DNA, 21 bp, synthetic construct
  misc_feature 20..21: note = dTdT
  source 1..21: mol_type = other DNA
  misc_feature 1..19: note = RNA
tttcatcagtcctgagcactt

SEQ ID NO: 114 - RNA, 21 nt, synthetic construct
  source 1..21: mol_type = other RNA
gtcaactgtggagcaacactt

SEQ ID NO: 115 - RNA, 21 nt, synthetic construct
  source 1..21: mol_type = other RNA
gtgttgctccacagttgactt

SEQ ID NO: 116 - DNA, 21 bp, synthetic construct
  source 1..21: mol_type = other DNA
  misc_feature 20..21: note = dTdT
  misc_feature 1..19: note = RNA
gcaacaacgccatctatgatt

SEQ ID NO: 117 - DNA, 21 bp, synthetic construct
  source 1..21: mol_type = other DNA
  misc_feature 20..21: note = dTdT
  misc_feature 1..19: note = RNA
tcatagatggcgttgttgctt

SEQ ID NO: 118 - RNA, 23 nt, synthetic construct
  source 1..23: mol_type = other RNA
gcaagacgttgtttgaaattatt

SEQ ID NO: 119 - RNA, 23 nt, synthetic construct
  source 1..23: mol_type = other RNA
taatttcaaacaacgtcttgctt

SEQ ID NO: 120 - RNA, 25 nt, synthetic construct
  source 1..25: mol_type = other RNA
cagcaagacgttgtttgaaattatt

SEQ ID NO: 121 - RNA, 25 nt, synthetic construct
  source 1..25: mol_type = other RNA
taatttcaaacaacgtcttgctgtt

SEQ ID NO: 122 - RNA, 21 nt, synthetic construct
  source 1..21: mol_type = other RNA
caggatggtaaagactacatt

SEQ ID NO: 123 - RNA, 21 nt, synthetic construct
  source 1..21: mol_type = other RNA
tgtagtctttaccatcctgtt

SEQ ID NO: 124 - DNA, 23 bp, synthetic construct
  source 1..23: mol_type = other DNA
gtcaacatcagtctgataagcta

SEQ ID NO: 125 - DNA, 22 bp, synthetic construct
  source 1..22: mol_type = other DNA
tcaacatcagtctgataagcta

SEQ ID NO: 126 - DNA, 23 bp, synthetic construct
  source 1..23: mol_type = other DNA
gctgagagtgtaggatgtttaca

SEQ ID NO: 127 - DNA, 22 bp, synthetic construct
  source 1..22: mol_type = other DNA
catcaccaccagagccaacgtc

SEQ ID NO: 128 - DNA, 45 bp, synthetic construct
  source 1..45: mol_type = other DNA
ggttgcatgccgtggggaggggggtgggttttatagcgtactcag

SEQ ID NO: 129 - DNA, 15 bp, synthetic construct
  source 1..15: mol_type = other DNA
ccctcctacataggg

SEQ ID NO: 130 - RNA, 15 nt, synthetic construct
  source 1..15: mol_type = other RNA
ccctcctacataggg

SEQ ID NO: 131 - DNA, 26 bp, synthetic construct
  source 1..26: mol_type = other DNA
ggtggtggtggttgtggtggtggtgg

SEQ ID NO: 132 - RNA, 26 nt, synthetic construct
  source 1..26: mol_type = other RNA
ggtggtggtggttgtggtggtggtgg

SEQ ID NO: 133 - RNA, 48 nt, synthetic construct
  source 1..48: mol_type = other RNA
attctgaaccgtgtgcagcaccacgctgcacacggttcagaatacaca

SEQ ID NO: 134 - DNA, 72 bp, synthetic construct
  source 1..72: mol_type = other DNA
ggcaggaagacaaacaagcttggcggcgggaaggtgtttaaattcccgggtctgcgtggtctgtggtgctgt

SEQ ID NO: 135 - DNA, 25 bp, synthetic construct
  source 1..25: mol_type = other DNA
acctggggagtattggggaggaagg

SEQ ID NO: 136 - DNA, 27 bp, synthetic construct
  source 1..27: mol_type = other DNA
gggaggacgatgcggaggaagggtagg

SEQ ID NO: 137 - DNA, 45 bp, synthetic construct
  source 1..45: mol_type = other DNA
cggggaaagtcacggggggtttcagatgttctgatcggtgtggag

SEQ ID NO: 138 - DNA, 15 bp, synthetic construct
  source 1..15: mol_type = other DNA
ccagatagtccctgg

SEQ ID NO: 139 - DNA, 24 bp, synthetic construct
  source 1..24: mol_type = other DNA
gataacgggcacgaattcggagtg

SEQ ID NO: 140 - RNA, 50 nt, synthetic construct
  source 1..50: mol_type = other RNA
agtgcaagacgttcgcagattagcgaaaagagggtctcattgactagtac

SEQ ID NO: 141 - RNA, 31 nt, synthetic construct
  source 1..31: mol_type = other RNA
ggtggaagagggatgggccgacgtgccgcat

SEQ ID NO: 142 - DNA, 62 bp, synthetic construct
  source 1..62: mol_type = other DNA
tccctacggcgctaacgatggtgaaaatgggcctagggtggacggtgccaccgtgctacaac

SEQ ID NO: 143 - DNA, 50 bp, synthetic construct
  source 1..50: mol_type = other DNA
atcaggctggatggtagctcggtcggggtgggtgggttggcaagtctgat

SEQ ID NO: 144 - DNA, 40 bp, synthetic construct
  source 1..40: mol_type = other DNA
agtctgttggaccgaatcccgtggacgcaccctttggacg

SEQ ID NO: 145 - DNA, 36 bp, synthetic construct
  source 1..36: mol_type = other DNA
cccacgtctgcgcttagctcctgggcctggatgggc

SEQ ID NO: 146 - RNA, 38 nt, synthetic construct
  source 1..38: mol_type = other RNA
tgactcctctgacagcctaatttctcccgattaccctg

SEQ ID NO: 147 - DNA, 40 bp, synthetic construct
  source 1..40: mol_type = other DNA
ccagtagccataccggtttgtggatggggtgtatgcgagt

SEQ ID NO: 148 - DNA, 40 bp, synthetic construct
  source 1..40: mol_type = other DNA
ctaggatccccactcaccatctctcagcttgcttcctagc

SEQ ID NO: 149 - RNA, 40 nt, synthetic construct
  source 1..40: mol_type = other RNA
ctaggatccccactcaccatctctcagcttgcttcctagc

SEQ ID NO: 150 - DNA, 18 bp, synthetic construct
  source 1..18: mol_type = other DNA
ttaacttattcgaccata

SEQ ID NO: 151 - DNA, 71 bp, synthetic construct
  source 1..71: mol_type = other DNA
tcgcgcgagtcgtctggggaaccatcgagttacaccgaccttctatgtgcggccccccgcatcgtcctccc

SEQ ID NO: 152 - DNA, 78 bp, synthetic construct
  source 1..78: mol_type = other DNA
accttggctgtcgtgttgtaggtggtttgctgcggtgggctcaagaagaaagcgcaaagaggtcagtggtcagagcgt

SEQ ID NO: 153 - DNA, 78 bp, synthetic construct
  source 1..78: mol_type = other DNA
accttggctgtcgtgttgtggggtgtcgtatctttcgtgtcttattattttctaggtggaggtcagtggtcagagcgt

SEQ ID NO: 154 - DNA, 25 bp, synthetic construct
  source 1..25: mol_type = other DNA
ccaacgagtaggcgatagcgcgtgg

SEQ ID NO: 155 - DNA, 50 bp, synthetic construct
  source 1..50: mol_type = other DNA
agagacgatgcggccaacgagtaggcgatagcgcgtggcagagcgtcgct

SEQ ID NO: 156 - DNA, 27 bp, synthetic construct
  source 1..27: mol_type = other DNA
gccaacgagtaggcgatagcgcgtggc

SEQ ID NO: 157 - DNA, 34 bp, synthetic construct
  source 1..34: mol_type = other DNA
ccactgcgggggtctatacgtgaggaagaagtgg

SEQ ID NO: 158 - DNA, 61 bp, synthetic construct
  source 1..61: mol_type = other DNA
tgcgtgtgtagtgtgtgtcgtttctcctttttttggttgctgctcttagggatttgggcgg

SEQ ID NO: 159 - DNA, 59 bp, synthetic construct
  source 1..59: mol_type = other DNA
tgcgtgtgtagtgtgtctgttctcctttttttggttgctgctcttagggatttgggcgg

SEQ ID NO: 160 - RNA, 25 nt, synthetic construct
  source 1..25: mol_type = other RNA
tgagccctgttcgacaggaggctca

SEQ ID NO: 161 - RNA, 51 nt, synthetic construct
  source 1..51: mol_type = other RNA
gggaggacgatgcggtttggggttttcccgtgccccagacgactcgcccga

SEQ ID NO: 162 - DNA, 87 bp, synthetic construct
  source 1..87: mol_type = other DNA
tctcggacgcgtgtggtcggccgagtggcccacggtagaagggttagaactgctggttggtgaatctcgctgcctggccctagagtg

SEQ ID NO: 163 - DNA, 30 bp, synthetic construct
  source 1..30: mol_type = other DNA
ccaaggcctgcaagggaaccaaggacacag

SEQ ID NO: 164 - DNA, 35 bp, synthetic construct
  source 1..35: mol_type = other DNA
gtggattgttgtgttctgttggtttttgtgttgtc

SEQ ID NO: 165 - DNA, 59 bp, synthetic construct
  source 1..59: mol_type = other DNA
tgcgtgtgtagtgtgtctgttttttatcttcttttatctactcttagggatttgggcgg

SEQ ID NO: 166 - DNA, 40 bp, synthetic construct
  source 1..40: mol_type = other DNA
tatgtgggtgggtgggcggttatgctgagtcagccttgct

SEQ ID NO: 167 - DNA, 76 bp, synthetic construct
  source 1..76: mol_type = other DNA
atccagagtgacgcagcatatgtgggtgggtgggcggttatgctgagtcagccttgcttggacacggtggcttagt

SEQ ID NO: 168 - RNA, 102 nt, synthetic construct
  source 1..102: mol_type = other RNA
gggagagaggaagagggatggggattagaccataggctcccaaccccccccgggagagaggaagagggatggggattagaccataggctcccaacccccggg

SEQ ID NO: 169 - DNA, 57 bp, synthetic construct
  source 1..57: mol_type = other DNA
taccagtgcgatgctcagcacgcttataggggctggacaaaattctacccagccttt

SEQ ID NO: 170 - DNA, 32 bp, synthetic construct
  source 1..32: mol_type = other DNA
tacgtgaatctcgtacgatactctgtaagcgt

SEQ ID NO: 171 - RNA, 90 nt, synthetic construct
  source 1..90: mol_type = other RNA
gggatggatccaagcttactggcatctggatttgcgcgtgccagaataaagagtataacgtgtgaatgggaagcttcgataggaattcgg

SEQ ID NO: 172 - DNA, 45 bp, synthetic construct
  source 1..45: mol_type = other DNA
gatcagttttccatgccagttggtattccgcgacagtttgatctc

SEQ ID NO: 173 - DNA, 35 bp, synthetic construct
  source 1..35: mol_type = other DNA
ggggccggggcaaggggggggtaccgtggtaggac

SEQ ID NO: 174 - DNA, 32 bp, synthetic construct
  source 1..32: mol_type = other DNA
caccccacctcgctcccgtgacactaatgcta

SEQ ID NO: 175 - DNA, 66 bp, synthetic construct
  source 1..66: mol_type = other DNA
tgcgtgtgtagtgtgtctgggctacatcgatgagctgcctagggtccctcttagggatttgggcgg

SEQ ID NO: 176 - DNA, 39 bp, synthetic construct
  source 1..39: mol_type = other DNA
gccttagtaacgtgctttgatgtcgattcgacaggaggc

SEQ ID NO: 177 - RNA, 39 nt, synthetic construct
  source 1..39: mol_type = other RNA
gccttagtaacgtgctttgatgtcgattcgacaggaggc

SEQ ID NO: 178 - RNA, 53 nt, synthetic construct
  source 1..53: mol_type = other RNA
tgccgctataatgcacggatttaatcgccgtagaaaagcatgtcaaagccgtt

SEQ ID NO: 179 - RNA, 19 nt, synthetic construct
  source 1..19: mol_type = other RNA
gcgactggttacccggtcg

SEQ ID NO: 180 - DNA, 48 bp, synthetic construct
  source 1..48: mol_type = other DNA
cactacagaggttgcgtctgtcccacgttgtcatggggggttggcctg

SEQ ID NO: 181 - DNA, 31 bp, synthetic construct
  source 1..31: mol_type = other DNA
gacaaacgggggaagatttgacgtcgacgac

SEQ ID NO: 182 - DNA, 47 bp, synthetic construct
  source 1..47: mol_type = other DNA
gcaggtccactgcgggggtctatacgtgaggaagaagtgggcaggtc

SEQ ID NO: 183 - RNA, 36 nt, synthetic construct
  source 1..36: mol_type = other RNA
gggatactagggcattaatgttaccagtgtagtccc

SEQ ID NO: 184 - RNA, 37 nt, synthetic construct
  source 1..37: mol_type = other RNA
gggaaactagggcgttaacgtgaccagtgtttctcga

SEQ ID NO: 185 - RNA, 35 nt, synthetic construct
  source 1..35: mol_type = other RNA
gggaaactagggcgttaacgtgaccagtgtttccc

SEQ ID NO: 186 - RNA, 56 nt, synthetic construct
  source 1..56: mol_type = other RNA
gggcgacctctccgtactgacctacagagcgacatactagtgtatccagatcgccc

SEQ ID NO: 187 - DNA, 21 bp, synthetic construct
  source 1..21: mol_type = other DNA
tgggggttgaggctaagccga

SEQ ID NO: 188 - DNA, 31 bp, synthetic construct
  source 1..31: mol_type = other DNA
ccgctcgagctagtctgacaaagagaaacac

SEQ ID NO: 189 - DNA, 21 bp, synthetic construct
  source 1..21: mol_type = other DNA
aacggagtgtggctaactcga

SEQ ID NO: 190 - DNA, 37 bp, synthetic construct
  source 1..37: mol_type = other DNA
taacgctgaccttagctgcatggctttacatgttcca

SEQ ID NO: 191 - DNA, 20 bp, synthetic construct
  source 1..20: mol_type = other DNA
gcagaggtgaagcgaagtcg

SEQ ID NO: 192 - DNA, 40 bp, synthetic construct
  source 1..40: mol_type = other DNA
cacagcgaacagcggcggacataatagtgcttactacgac

SEQ ID NO: 193 - DNA, 34 bp, synthetic construct
  source 1..34: mol_type = other DNA
agccgcgaggggagggatagggtagggcgcggct

SEQ ID NO: 194 - RNA, 34 nt, synthetic construct
  source 1..34: mol_type = other RNA
agccgcgaggggagggatagggtagggcgcggct

SEQ ID NO: 195 - DNA, 81 bp, synthetic construct
  source 1..81: mol_type = other DNA
gggagctcagaataaacgctcaaagggtcaagctgattacactttgtccactattgggtccttcgacatgaggcccggatc

SEQ ID NO: 196 - DNA, 81 bp, synthetic construct
  source 1..81: mol_type = other DNA
gggagctcagaataaacgctcaaggctaacagcacgcaacgggggggagtaatcgtgtctgttcgacatgaggcccggatc

SEQ ID NO: 197 - RNA, 49 nt, synthetic construct
  source 1..49: mol_type = other RNA
cagcgaaagttgcgtatgggtcacatcgcaggcacatgtcatctgggcg

SEQ ID NO: 198 - RNA, 79 nt, synthetic construct
  source 1..79: mol_type = other RNA
gaattccgcgtgtgccagcgaaagttgcgtatgggccacatcgcaggcacatgtcatctgggcggtccgttcgggatcc

SEQ ID NO: 199 - DNA, 23 bp, synthetic construct
  source 1..23: mol_type = other DNA
ggaaaaaattttttaaaaaaccc

SEQ ID NO: 200 - DNA, 54 bp, synthetic construct
  source 1..54: mol_type = other DNA
gggccgtcgaacacgagcatggtgcgtggacctaggatgacctgagtactgtcc

SEQ ID NO: 201 - DNA, 63 bp, synthetic construct
  source 1..63: mol_type = other DNA
ccgcccaaatccctaagagaagactgtaatgacatcaaaccagacacacacactacacacgca

SEQ ID NO: 202 - RNA, 79 nt, synthetic construct
  source 1..79: mol_type = other RNA
ggaggacgatgcggaaaaagcaacagggtgctccatgcgcatggaacctgcgcgcagacgactcgctgaggatccgaga

SEQ ID NO: 203 - RNA, 40 nt, synthetic construct
  source 1..40: mol_type = other RNA
aaaaagcaacagggtgctccatgcgcatggaacctgcgcg

SEQ ID NO: 204 - DNA, 30 bp, synthetic construct
  source 1..30: mol_type = other DNA
cttggatcaccatagtcgctagtcgaggct

SEQ ID NO: 205 - DNA, 24 bp, synthetic construct
  source 1..24: mol_type = other DNA
gcggcatcctatcacgcattgacc

SEQ ID NO: 206 - RNA, 70 nt, synthetic construct
  source 1..70: mol_type = other RNA
gggagagagatataagggcctcctgatacccgctgctatctggaccgatcccattaccaaattctctccc

SEQ ID NO: 207 - DNA, 60 bp, synthetic construct
  source 1..60: mol_type = other DNA
atccagagtgacgcagcatattagtacggcttaaccccatggtggacacggtggcttagt

SEQ ID NO: 208 - DNA, 25 bp, synthetic construct
  source 1..25: mol_type = other DNA
gcagttgatcctttggataccctgg

SEQ ID NO: 209 - DNA, 25 bp, synthetic construct
  source 1..25: mol_type = other DNA
gaagtgaaaatgacagaacacaaca

SEQ ID NO: 210 - DNA, 88 bp, synthetic construct
  source 1..88: mol_type = other DNA
aaccgcccaaatctctaagagtcggactgcaacctatgctatcgttgatgtctgtccaagcaacacagacacactacacacacgcaca

SEQ ID NO: 211 - DNA, 19 bp, synthetic construct
  source 1..19: mol_type = other DNA
aatgacagaacacaacatt

SEQ ID NO: 212 - RNA, 25 nt, synthetic construct
  source 1..25: mol_type = other RNA
gcagttgatcctttggataccctgg

SEQ ID NO: 213 - DNA, 80 bp, synthetic construct
  source 1..80: mol_type = other DNA
agcagcacagaggtcagatgcttggttccaccgtactgactgtagtaaaatctgatcactcctatgcgtgctaccgtgaa

SEQ ID NO: 214 - DNA, 80 bp, synthetic construct
  source 1..80: mol_type = other DNA
agcagcacagaggtcagatgtagtcggtcttcttgtttgaaactgctaattttgaaaaaacctatgcgtgctaccgtgaa

SEQ ID NO: 215 - DNA, 80 bp, synthetic construct
  source 1..80: mol_type = other DNA
agcagcacagaggtcagatgatataaccttaataaataaaatataaattatttaatcttacctatgcgtgctaccgtgaa

SEQ ID NO: 216 - RNA, 50 nt, synthetic construct
  source 1..50: mol_type = other RNA
gggagaatagtcaacaaatcgtttggggcgacttctccttcctttctccc

SEQ ID NO: 217 - DNA, 40 bp, synthetic construct
  source 1..40: mol_type = other DNA
gattgagtagatagtggttctgtacgtagtgaaagagtgg

SEQ ID NO: 218 - DNA, 94 bp, synthetic construct
  source 1..94: mol_type = other DNA
caagttgctcgtcgcgatacgtttggttggtgtggttggcagtatcgcaggtccaagttgctcgtcgcgatacaacggagtgtggctaactcga

SEQ ID NO: 219 - DNA, 46 bp, synthetic construct
  source 1..46: mol_type = other DNA
caagttgctcgtcgcgatacgtttggttggtgtggttggcagtatc

SEQ ID NO: 220 - DNA, 39 bp, synthetic construct
  source 1..39: mol_type = other DNA
tcacacggacctctctctacattaattgcgcatttcgtt

SEQ ID NO: 221 - DNA, 58 bp, synthetic construct
  source 1..58: mol_type = other DNA
gctggatgttcatgctggcaaaattccttaggggcaccgttactttgacacatccagc

SEQ ID NO: 222 - DNA, 58 bp, synthetic construct
  source 1..58: mol_type = other DNA
gctggatgtcgcttacgacaatattccttaggggcaccgctacattgacacatccagc

SEQ ID NO: 223 - DNA, 58 bp, synthetic construct
  source 1..58: mol_type = other DNA
gctggatgtcaccggattgtcggacatcggattgtctgagtcatatgacacatccagc

SEQ ID NO: 224 - DNA, 58 bp, synthetic construct
  source 1..58: mol_type = other DNA
gctggatgttgacctttacagatcggattctgtggggcgttaaactgacacatccagc

SEQ ID NO: 225 - DNA, 80 bp, synthetic construct
  source 1..80: mol_type = other DNA
gggaggacgatgcggcagtctgcatcgtaggaatcgccaccgtatactttcccaccagacgactcgctgaggatccgaga

SEQ ID NO: 226 - RNA, 80 nt, synthetic construct
  source 1..80: mol_type = other RNA
gggaggacgatgcggcagtctgcatcgtaggaatcgccaccgtatactttcccaccagacgactcgctgaggatccgaga

SEQ ID NO: 227 - DNA, 39 bp, synthetic construct
  misc_feature 28: note = RNA U
  source 1..39: mol_type = other DNA
  misc_feature 1..27: note = DNA
  misc_feature 29..39: note = DNA
cagtctgcatcgtaggattagccaccgtatctttcccac

SEQ ID NO: 228 - RNA, 69 nt, synthetic construct
  source 1..69: mol_type = other RNA
gggaggacgatgcggcagtctgcatcgtaggaatcgccaccgtatactttcccaccagacgactcgctg

SEQ ID NO: 229 - RNA, 40 nt, synthetic construct
  source 1..40: mol_type = other RNA
cagtctgcatcgtaggaatcgccaccgtatactttcccac

SEQ ID NO: 230 - RNA, 54 nt, synthetic construct
  source 1..54: mol_type = other RNA
gggatgcggaaaaaagaacacttccgattagggcccaccctaacggccgcagac

SEQ ID NO: 231 - DNA, 39 bp, synthetic construct
  source 1..39: mol_type = other DNA
gggaggacgatgcggatcagccatgtttacgtcactcct

SEQ ID NO: 232 - DNA, 48 bp, synthetic construct
  source 1..48: mol_type = other DNA
gcgttttcgcttttgcgttttgggtcatctgcttacgatagcaatgct

SEQ ID NO: 233 - RNA, 39 nt, synthetic construct
  source 1..39: mol_type = other RNA
gggaggacgatgcggatcagccatgtttacgtcactcct

SEQ ID NO: 234 - RNA, 43 nt, synthetic construct
  source 1..43: mol_type = other RNA
gggaccgaaaaagacctgacttctatactaagtctacgttccc

SEQ ID NO: 235 - DNA, 33 bp, synthetic construct
  source 1..33: mol_type = other DNA
tgtcgtggggcatcgagtaaatgcaattcgaca

SEQ ID NO: 236 - RNA, 33 nt, synthetic construct
  source 1..33: mol_type = other RNA
tgtcgtggggcatcgagtaaatgcaattcgaca

SEQ ID NO: 237 - DNA, 35 bp, synthetic construct
  source 1..35: mol_type = other DNA
caggctacggcacgtagagcatcaccatgatcctg

SEQ ID NO: 238 - DNA, 40 bp, synthetic construct
  source 1..40: mol_type = other DNA
aacaacgtataacaatgcccacgtcaccagagtactatgg

SEQ ID NO: 239 - DNA, 33 bp, synthetic construct
  source 1..33: mol_type = other DNA
gccccagttatgctttccccctctgtctctttg

SEQ ID NO: 240 - DNA, 31 bp, synthetic construct
  source 1..31: mol_type = other DNA
atcgcccgcagcacccatttgtttttttttg

SEQ ID NO: 241 - DNA, 45 bp, synthetic construct
  source 1..45: mol_type = other DNA
acgggccacatcaactcattgatagacaatgcgtccactgcccgt

SEQ ID NO: 242 - DNA, 45 bp, synthetic construct
  source 1..45: mol_type = other DNA
tgcccgcacatcaactcattgatagacaatgcgtccactcgggca

SEQ ID NO: 243 - DNA, 45 bp, synthetic construct
  source 1..45: mol_type = other DNA
tgcccgcacatcaactcattgatagacaatgcgtccactacgggc

SEQ ID NO: 244 - DNA, 45 bp, synthetic construct
  source 1..45: mol_type = other DNA
cgggcacacatcaactcattgatagacaatgcgtccactgcccgt

SEQ ID NO: 245 - DNA, 45 bp, synthetic construct
  source 1..45: mol_type = other DNA
gttggtcacatcaactcattgatagacaatgcgtccactaccaac

SEQ ID NO: 246 - DNA, 41 bp, synthetic construct
  source 1..41: mol_type = other DNA
gggccacatcaactcattgatagacaatgcgtccactgccc

SEQ ID NO: 247 - DNA, 45 bp, synthetic construct
  source 1..45: mol_type = other DNA
tggttgcacatcaactcattgatagacaatgcgtccactcaacca

SEQ ID NO: 248 - DNA, 33 bp, synthetic construct
  source 1..33: mol_type = other DNA
tacaggttctggggggtgggtggggaacctgtt

SEQ ID NO: 249 - DNA, 38 bp, synthetic construct
  source 1..38: mol_type = other DNA
ctacgagacgaacttatgcgtaataatgactgtcgtag

SEQ ID NO: 250 - DNA, 75 bp, synthetic construct
  source 1..75: mol_type = other DNA
gacgatagcggtgacggcacagacggtacagttcccgtccctgcactacacgtatgccgcttccgtccgtcgctc

SEQ ID NO: 251 - DNA, 75 bp, synthetic construct
  source 1..75: mol_type = other DNA
gagcgacggacggaagcggcatacgtgtagtgcagggacgggaactgtaccgtctgtgccgtcaccgctatcgtc

SEQ ID NO: 252 - DNA, 71 bp, synthetic construct
  source 1..71: mol_type = other DNA
ggatcctatgacgcattgacccgctgcctctactgaggctgtgtcagtgtgcggctcggactgttgaattc

SEQ ID NO: 253 - DNA, 55 bp, synthetic construct
  source 1..55: mol_type = other DNA
agcggtgacggcacagacggtacagttcccgtccctgcactacacgtatgccgct

SEQ ID NO: 254 - DNA, 40 bp, synthetic construct
  source 1..40: mol_type = other DNA
accgacagtgaaggactcagcgaactctcagactcggttc

SEQ ID NO: 255 - DNA, 41 bp, synthetic construct
  source 1..41: mol_type = other DNA
atctaactgctgcgccgccgggaaaatactgtacggttaga

SEQ ID NO: 256 - DNA, 47 bp, synthetic construct
  source 1..47: mol_type = other DNA
catgcggagtagagcgagcccagatagtccctggttatttccttagg

SEQ ID NO: 257 - DNA, 40 bp, synthetic construct
  source 1..40: mol_type = other DNA
gatctctctctgccctaagtccgcacccgtgcttccctgt

SEQ ID NO: 258 - DNA, 15 bp, synthetic construct
  source 1..15: mol_type = other DNA
ggttggtgtggttgg

SEQ ID NO: 259 - DNA, 29 bp, synthetic construct
  source 1..29: mol_type = other DNA
agtccgtggtagggcaggttggggtgact

SEQ ID NO: 260 - DNA, 14 bp, synthetic construct
  source 1..14: mol_type = other DNA
gcgtggtaccacgc

SEQ ID NO: 261 - RNA, 14 nt, synthetic construct
  source 1..14: mol_type = other RNA
gcgtggtaccacgc

SEQ ID NO: 262 - DNA, 14 bp, synthetic construct
  source 1..14: mol_type = other DNA
gcgtggtcacacgc

SEQ ID NO: 263 - RNA, 14 nt, synthetic construct
  source 1..14: mol_type = other RNA
gcgtggtcacacgc

SEQ ID NO: 264 - DNA, 74 bp, synthetic construct
  source 1..74: mol_type = other DNA
gcggcgcccacgagcgttcgcgtggtcacacgcgttccgccctcctacatagggcgcatagccgtgggcgccgc

SEQ ID NO: 265 - DNA, 34 bp, synthetic construct
  source 1..34: mol_type = other DNA
cctgcacttggcttggatttcagaagggagaccc

SEQ ID NO: 266 - DNA, 33 bp, synthetic construct
  source 1..33: mol_type = other DNA
ctgcacttggcttggatttcagaagggagaccc

SEQ ID NO: 267 - RNA, 34 nt, synthetic construct
  source 1..34: mol_type = other RNA
cctgcacttggcttggatttcagaagggagaccc

SEQ ID NO: 268 - DNA, 39 bp, synthetic construct
  source 1..39: mol_type = other DNA
agtccattttattcctgaatatttgttaacctcatggac

SEQ ID NO: 269 - DNA, 60 bp, synthetic construct
  source 1..60: mol_type = other DNA
acattgctgcgtgatcgcctcacatgggtttgtctggtcgatttggaggtggtgggtggc

SEQ ID NO: 270 - RNA, 61 nt, synthetic construct
  source 1..61: mol_type = other RNA
gggagaggaccagtagccactatggtgttggagctagcggcagagcgtcgcggtccctccc

SEQ ID NO: 271 - RNA, 61 nt, synthetic construct
  source 1..61: mol_type = other RNA
gggagaggaccagtactggtagttctctgtgcgactcctacagagcgtcgcggtccctccc

SEQ ID NO: 272 - RNA, 38 nt, synthetic construct
  source 1..38: mol_type = other RNA
aagcaacacttagtcgcgattgatacgtgcgcagtcat

SEQ ID NO: 273 - RNA, 79 nt, synthetic construct
  source 1..79: mol_type = other RNA
ggaggacgatgcggggaagcaacacttagtcgcgattgatacgtgcgcagtcatcagacgactcgctgaggatccgaga

SEQ ID NO: 274 - DNA, 33 bp, synthetic construct
  source 1..33: mol_type = other DNA
gcggccgataaggtctttccaagcgaacgaaaa

SEQ ID NO: 275 - DNA, 41 bp, synthetic construct
  source 1..41: mol_type = other DNA
gcgccactacaggggagctgccattcgaataggtgggccgc

SEQ ID NO: 276 - DNA, 74 bp, synthetic construct
  source 1..74: mol_type = other DNA
cgctcgatagatcgagcttcgctcgatgtggtgttgtgggggcttgtattggtcgatcacgctctagagcactg

SEQ ID NO: 277 - DNA, 26 bp, synthetic construct
  source 1..26: mol_type = other DNA
tggtgggggtggacgggccgggtaga

SEQ ID NO: 278 - RNA, 23 nt, synthetic construct
  source 1..23: mol_type = other RNA
atgcagtttgagaagtcgcgcat

SEQ ID NO: 279 - DNA, 25 bp, synthetic construct
  source 1..25: mol_type = other DNA
ggtgggggtggacgggccgggtaga

SEQ ID NO: 280 - RNA, 27 nt, synthetic construct
  source 1..27: mol_type = other RNA
cggaatcagtgaatgcttatacatccg

SEQ ID NO: 281 - DNA, 25 bp, synthetic construct
  source 1..25: mol_type = other DNA
tgtgggggtggactgggtgggtacc

SEQ ID NO: 282 - DNA, 25 bp, synthetic construct
  source 1..25: mol_type = other DNA
tgtgggggtggacgggccgggtaga

SEQ ID NO: 283 - DNA, 95 bp, synthetic construct
  source 1..95: mol_type = other DNA
ataccagcttattcaattggacacggcaaaggggtatagcctaccggaccgtgaacatggaatggtgtgctgcgtggagatagtaagtgcaatct

SEQ ID NO: 284 - DNA, 59 bp, synthetic construct
  source 1..59: mol_type = other DNA
ggacacggcaaaggggtatagcctaccggaccgtgaacatggaatggtgtgctgcgtgg

SEQ ID NO: 285 - DNA, 39 bp, synthetic construct
  source 1..39: mol_type = other DNA
agggaatcttgcctagggagggagtagcgaaagggctca

SEQ ID NO: 286 - RNA, 96 nt, synthetic construct
  source 1..96: mol_type = other RNA
gggagagaggaagagggatgggcgaccgaacgtgcccttcaaagccgttcactaaccagtggcataacccagaggtcgatagtactggatcccccc

SEQ ID NO: 287 - DNA, 56 bp, synthetic construct
  source 1..56: mol_type = other DNA
actcatagggttaggggctgctggccagatactcagatggtagggttactatgagc

SEQ ID NO: 288 - DNA, 40 bp, synthetic construct
  source 1..40: mol_type = other DNA
aacagagggacaaacgggggaagatttgacgtcgacgaca

SEQ ID NO: 289 - DNA, 52 bp, synthetic construct
  source 1..52: mol_type = other DNA
cgacccggcacaaacccagaaccatatacacgatcattagtctcctgggccg

SEQ ID NO: 290 - DNA, 53 bp, synthetic construct
  source 1..53: mol_type = other DNA
atccagagtgacgcagcaccaccaccgtacaattttttcattacctactcggc

SEQ ID NO: 291 - DNA, 45 bp, synthetic construct
  source 1..45: mol_type = other DNA
cccatcaatgttacgacccgctagggctgctgtgccatcgggtaa

SEQ ID NO: 292 - DNA, 74 bp, synthetic construct
  source 1..74: mol_type = other DNA
agaattcagtcggacagcgaagtagttttccttctaacctaagaacccgcggcagtttaatgtagatggacgaa

SEQ ID NO: 293 - DNA, 45 bp, synthetic construct
  source 1..45: mol_type = other DNA
gcatggggtttcggcgtttcgtctatcttgtttctgttagcgtct

SEQ ID NO: 294 - DNA, 57 bp, synthetic construct
  source 1..57: mol_type = other DNA
tgccactacagctggttcggtttggtgacttcgttcttcgttgtggtgcttagtggc

SEQ ID NO: 295 - DNA, 21 bp, synthetic construct
  source 1..21: mol_type = other DNA
gcccacgagcgttccgggaga

SEQ ID NO: 296 - DNA, 21 bp, synthetic construct
  source 1..21: mol_type = other DNA
ctcgcggccatagccgtgggc

SEQ ID NO: 297 - DNA, 64 bp, synthetic construct
  source 1..64: mol_type = other DNA
tgctgctgctgctgtttttacgggccacatcaactcattgatagacaatgcgtccactgcccgt

SEQ ID NO: 298 - DNA, 52 bp, synthetic construct
  source 1..52: mol_type = other DNA
tgctgctgctgctgttttttacaggttctggggggtgggtggggaacctgtt

SEQ ID NO: 299 - DNA, 45 bp, synthetic construct
  source 1..45: mol_type = other DNA
cgcggctcgcggctcgcggctcgcggccatagccgtgggcgtcgc

SEQ ID NO: 300 - RNA, 23 nt, synthetic construct
  source 1..23: mol_type = other RNA
tgtgacagataaggaacctgcag

SEQ ID NO: 301 - RNA, 19 nt, synthetic construct
  source 1..19: mol_type = other RNA
gctgcacacggttcagaat

SEQ ID NO: 302 - RNA, 23 nt, synthetic construct
  source 1..23: mol_type = other RNA
aattagataagactgctaaggca

SEQ ID NO: 303 - RNA, 21 nt, synthetic construct
  source 1..21: mol_type = other RNA
gcaggttccttatctgtcaca

SEQ ID NO: 304 - RNA, 19 nt, synthetic construct
  source 1..19: mol_type = other RNA
gcaggttccttatctgtca

SEQ ID NO: 305 - RNA, 23 nt, synthetic construct
  source 1..23: mol_type = other RNA
tgacagataaggaacctgcagtt

SEQ ID NO: 306 - DNA, 107 bp, synthetic construct
  source 1..107: mol_type = other DNA
tctcggacgcgtgtggtcggccgagtggcccacggtagaagggttagaactgctggttggtgaatctcgctgcctggccctagagtgttttttgccaccgtgctaca

SEQ ID NO: 307 - DNA, 59 bp, synthetic construct
  source 1..59: mol_type = other DNA
accgacagtgaaggactcagcgaactctcagactcggttctttttcacggccgcgccga

SEQ ID NO: 308 - RNA, 65 nt, synthetic construct
  source 1..65: mol_type = other RNA
agtgcaagacgttcgcagattagcgaaaagagggtctcattgactagtactcagcagcagcagca

SEQ ID NO: 309 - DNA, 60 bp, synthetic construct
  source 1..60: mol_type = other DNA
tcgtcgttttgtcgttttgtcgtttttttgcgacgcccacgagcgttccgggagaggagc

SEQ ID NO: 310 - DNA, 66 bp, synthetic construct
  source 1..66: mol_type = other DNA
tacgtgaatctcgtacgatactctgtaagcgttttttgctcctctcccggttcgccgcgagccgcg

SEQ ID NO: 311 - DNA, 76 bp, synthetic construct
  source 1..76: mol_type = other DNA
aacaacgtataacaatgcccacgtcaccagagtactatggtttttcgcggctcgcggccatagccgtgggcgtcgc

SEQ ID NO: 312 - DNA, 96 bp, synthetic construct
  source 1..96: mol_type = other DNA
tgcgtgtgtagtgtgtctgttttttatcttcttttatctactcttagggatttgggcggagcgaagcgacgcccacgagcgttccgggagaggagc

SEQ ID NO: 313 - DNA, 69 bp, synthetic construct
  source 1..69: mol_type = other DNA
tacgtgaatctcgtacgatactctgtaagcgttgtgacaggctcctctcccggttcgccgcgagccgcg

SEQ ID NO: 314 - DNA, 75 bp, synthetic construct
  source 1..75: mol_type = other DNA
gccgcggggtgggtctagtgtggatgtttagggggcggctttttcgcggctcgcggccatagccgtgggcgtcgc

SEQ ID NO: 315 - DNA, 69 bp, synthetic construct
  source 1..69: mol_type = other DNA
  misc_feature 33..40: note = miR-126
  misc_feature 1..32: note = DNA
  misc_feature 41..69: note = DNA
tacgtgaatctcgtacgatactctgtaagcgttcgtaccggctcctctcccggttcgccgcgagccgcg

SEQ ID NO: 316 - DNA, 89 bp, synthetic construct
  misc_feature 1..51: note = BCMA RNA aptamer
  source 1..89: mol_type = other DNA
  misc_feature 52..58: note = miR-126
  misc_feature 59..89: note = DNA
agtgcaagacgttcgcagattagcgaaaagagggtctcattgactagtactcgtaccggcgacgcccacgagcgttccgggagaggagc

SEQ ID NO: 317 - DNA, 69 bp, synthetic construct
  source 1..69: mol_type = other DNA
tacgtgaatctcgtacgatactctgtaagcgtggaagtgtgctcctctcccggttcgccgcgagccgcg

SEQ ID NO: 318 - DNA, 80 bp, synthetic construct
  source 1..80: mol_type = other DNA
agccgcggggtgggtctagtgtggatgtttagggggcggcttgtgacagcgcggctcgcggccatagccgtgggcgtcgc

SEQ ID NO: 319 - DNA, 76 bp, synthetic construct
  source 1..76: mol_type = other DNA
taacgctgaccttagctgcatggctttacatgttccagataagctgcgacgcccacgagcgttccgggagaggagc

SEQ ID NO: 320 - DNA, 79 bp, synthetic construct
  source 1..79: mol_type = other DNA
aacaacgtataacaatgcccacgtcaccagagtactatggtgtgacagcgcggctcgcggccatagccgtgggcgtcgc

SEQ ID NO: 321 - DNA, 64 bp, synthetic construct
  misc_feature 1..27: note = VEGF165 RNA aptamer
  source 1..64: mol_type = other DNA
  misc_feature 28..64: note = DNA
cggaatcagtgaatgcttatacatccgggaagtgtgctcctctcccggttcgccgcgagccgcg

SEQ ID NO: 322 - DNA, 77 bp, synthetic construct
  source 1..77: mol_type = other DNA
cacagcgaacagcggcggacataatagtgcttactacgacggaagtgtgctcctctcccggttcgccgcgagccgcg

SEQ ID NO: 323 - DNA, 56 bp, synthetic construct
  source 1..56: mol_type = other DNA
gcagaggtgaagcgaagtcgtttttgcgacgcccacgagcgttccgggagaggagc

SEQ ID NO: 324 - DNA, 83 bp, synthetic construct
  misc_feature 1..52: note = BCMA RNA aptamer and UU
  source 1..83: mol_type = other DNA
  misc_feature 53..83: note = DNA
agtgcaagacgttcgcagattagcgaaaagagggtctcattgactagtacttgcgacgcccacgagcgttccgggagaggagc

SEQ ID NO: 325 - DNA, 67 bp, synthetic construct
  source 1..67: mol_type = other DNA
tacgtgaatctcgtacgatactctgtaagcgtgtcgttgctcctctcccggttcgccgcgagccgcg

SEQ ID NO: 326 - DNA, 56 bp, synthetic construct
  source 1..56: mol_type = other DNA
ggtggtggtggttgtggtggtggtggtttttgcgcccacgagcgttccgggagagc

SEQ ID NO: 327 - DNA, 67 bp, synthetic construct
  misc_feature 1..41: note = FGF2 RNA aptamer and U
  source 1..67: mol_type = other DNA
  misc_feature 42..67: note = DNA
gggatactagggcattaatgttaccagtgtagtccctccctgctctcccggttcgccgccagccgcc

SEQ ID NO: 328 - DNA, 52 bp, synthetic construct
  source 1..52: mol_type = other DNA
gataagctgataagctgataagctggcggcaggcggccatagccgtgggcgc

SEQ ID NO: 329 - DNA, 76 bp, synthetic construct
  source 1..76: mol_type = other DNA
cacagcgaacagcggcggacataatagtgcttactacgactttttgcgacgcccacgagcgttccgggagaggagc

SEQ ID NO: 330 - DNA, 59 bp, synthetic construct
  source 1..59: mol_type = other DNA
ccaacgagtaggcgatagcgcgtggtttttgctcctctcccggttcgccgcgagccgcg

SEQ ID NO: 331 - DNA, 81 bp, synthetic construct
  source 1..81: mol_type = other DNA
acgggccacatcaactcattgatagacaatgcgtccactgcccgttttttcgcggctcgcggccatagccgtgggcgtcgc

SEQ ID NO: 332 - DNA, 54 bp, synthetic construct
  source 1..54: mol_type = other DNA
tacgtgaatctcgtacgatactctgtaagcgtttagcgaagccaccgtgctaca

SEQ ID NO: 333 - DNA, 47 bp, synthetic construct
  misc_feature 1..33: note = 1 to 25 is CD19 RNA aptamer, 26 to 33 is RNA type of AmiR-21
  source 1..47: mol_type = other DNA
  misc_feature 34..47: note = DNA
tgagccctgttcgacaggaggctcagataagctcacggccgcgccga

SEQ ID NO: 334 - DNA, 66 bp, synthetic construct
  misc_feature 1..50: note = BCMA RNA aptamer
  source 1..66: mol_type = other DNA
  misc_feature 51..60: note = DNA
agtgcaagacgttcgcagattagcgaaaagagggtctcattgactagtacaacagcagcagcagca

SEQ ID NO: 335 - DNA, 51 bp, synthetic construct
  source 1..51: mol_type = other DNA
tacgtgaatctcgtacgatactctgtaagcgttttttgccaccgtgctaca

SEQ ID NO: 336 - DNA, 64 bp, synthetic construct
  source 1..64: mol_type = other DNA
acgggccacatcaactcattgatagacaatgcgtccactgcccgttttttcacggccgcgccga

SEQ ID NO: 337 - DNA, 43 bp, synthetic construct
  source 1..43: mol_type = other DNA
tcgtcgttttgtcgttttgtcgtttttttcagcagcagcagca

SEQ ID NO: 338 - DNA, 46 bp, synthetic construct
  source 1..46: mol_type = other DNA
gccaacgagtaggcgatagcgcgtggctttttgccaccgtgctaca

SEQ ID NO: 339 - DNA, 68 bp, synthetic construct
  source 1..68: mol_type = other DNA
ccaacgagtaggcgatagcgcgtggtttgctcctctcccggttcgccgcgagcctcggcgcggccgtg

SEQ ID NO: 340 - DNA, 28 bp, synthetic construct
  source 1..28: mol_type = other DNA
ggctcgcggccatagccgtgggcgtcgc

SEQ ID NO: 341 - DNA, 44 bp, synthetic construct
  source 1..44: mol_type = other DNA
tcgtcgttttgtcgttttgtcgttttttttcagcagcagcagca

SEQ ID NO: 342 - DNA, 78 bp, synthetic construct
  source 1..78: mol_type = other DNA
acgggccacatcaactcattgatagacaatgcgtccactgcccgttttttggctcgcggccatagccgtgggcgtcgc

SEQ ID NO: 343 - DNA, 69 bp, synthetic construct
  source 1..69: mol_type = other DNA
tcgtcgttttgtcgttttgtcgtttttttgacgcccacgagcgttccgggagaggtgtagcacggtggc

SEQ ID NO: 344 - RNA, 23 nt, synthetic construct
  source 1..23: mol_type = other RNA
gtcaacatcagtctgataagcta

SEQ ID NO: 345 - RNA, 22 nt, synthetic construct
  source 1..22: mol_type = other RNA
tcaacatcagtctgataagcta

SEQ ID NO: 346 - DNA, 55 bp, synthetic construct
  source 1..55: mol_type = other DNA
tcgtcgttttgtcgttttgtcgtttttttgcggcgcccacgagcgttccgggagc

SEQ ID NO: 347 - DNA, 53 bp, synthetic construct
  source 1..53: mol_type = other DNA
tcgtcgttttgtcgttttgtcgtttttttgctcccggttcgccgccagccgcc

SEQ ID NO: 348 - DNA, 60 bp, synthetic construct
  source 1..60: mol_type = other DNA
tcgtcgttttgtcgttttgtcgtttttttggcggcaggcggccatagccgtgggcgccgc

SEQ ID NO: 349 - DNA, 53 bp, synthetic construct
  source 1..53: mol_type = other DNA
tccatgacgttcctgacgtttttgcgacgcccacgagcgttccgggagaggag

SEQ ID NO: 350 - DNA, 54 bp, synthetic construct
  source 1..54: mol_type = other DNA
tccatgacgttcctgacgtttttcgcggcacgcggccatagccgtgggcgtcgc

SEQ ID NO: 351 - DNA, 58 bp, synthetic construct
  source 1..58: mol_type = other DNA
ccaacgagtaggcgatagcgcgtggtttttctcctctcccggttcgccgcgagccgcg

SEQ ID NO: 352 - DNA, 59 bp, synthetic construct
  source 1..59: mol_type = other DNA
tcgtcgttttgtcgttttgtcgtttttttgcgacgcccacgagcgttccgggagaggag

SEQ ID NO: 353 - DNA, 60 bp, synthetic construct
  source 1..60: mol_type = other DNA
tcgtcgttttgtcgttttgtcgtttttttcgcggcacgcggccatagccgtgggcgtcgc

SEQ ID NO: 354 - DNA, 83 bp, synthetic construct
  source 1..83: mol_type = other DNA
tcgtcgttttgtcgttttgtcgtttcgtcgttttgtcgttttgtcgtttttttgcgacgcccacgagcgttccgggagaggag

SEQ ID NO: 355 - DNA, 84 bp, synthetic construct
  source 1..84: mol_type = other DNA
tcgtcgttttgtcgttttgtcgtttcgtcgttttgtcgttttgtcgtttttttcgcggcacgcggccatagccgtgggcgtcgc

SEQ ID NO: 356 - DNA, 61 bp, synthetic construct
  source 1..61: mol_type = other DNA
gcagttgatcctttggataccctggtttttcgcggcacgcggccatagccgtgggcgtcgc

SEQ ID NO: 357 - DNA, 66 bp, synthetic construct
  source 1..66: mol_type = other DNA
ccaacgagtaggcgatagcgcgtggtttttctcctctcccggttcgccgcgagccgcggataagct

SEQ ID NO: 358 - DNA, 61 bp, synthetic construct
  source 1..61: mol_type = other DNA
tcgtcgttttgtcgttttgtcgtttttttgcgacgcccacgagcgttccgggagaggagct

SEQ ID NO: 359 - DNA, 98 bp, synthetic construct
  source 1..98: mol_type = other DNA
ccaacgagtaggcgatagcgcgtggtttttgctcctctcccggttcgccgcgagccgcgtttttccactgcgggggtctatacgtgaggaagaagtgg

SEQ ID NO: 360 - DNA, 96 bp, synthetic construct
  misc_feature 66..96: note = CTLA-4 RNA aptamer
  source 1..96: mol_type = other DNA
  misc_feature 1..65: note = DNA
tcgtcgttttgtcgttttgtcgtttttttcgcggcacgcggccatagccgtgggcgtcgctttttggtggaagagggatgggccgacgtgccgcat

SEQ ID NO: 361 - DNA, 85 bp, synthetic construct
  source 1..85: mol_type = other DNA
tcgtcgttttgtcgttttgtcgtttcgtcgttttgtcgttttgtcgtttttttgcgacgcccacgagcgttccgggagaggagct

SEQ ID NO: 362 - DNA, 66 bp, synthetic construct
  misc_feature 1..49: note = CLTA-4 RNA aptamer
  source 1..66: mol_type = other DNA
  misc_feature 50..66: note = DNA
ggtggaagagggatgggccgacgtgccgcattttttgctcctctcccggttcgccgcgagccgcgt

SEQ ID NO: 363 - DNA, 83 bp, synthetic construct
  source 1..83: mol_type = other DNA
acgggccacatcaactcattgatagacaatgcgtccactgcccgttttttcgcggctcgcggctcatagccgtgggcgtcgct

SEQ ID NO: 364 - DNA, 75 bp, synthetic construct
  source 1..75: mol_type = other DNA
aacaacgtataacaatgcccacgtcaccagagtactatggatttcgcggctcgcggccatagccgtgggcgtcgc

SEQ ID NO: 365 - DNA, 49 bp, synthetic construct
  source 1..49: mol_type = other DNA
tcgtcgttttgtcgttttgtcgttttttgcccacgagcgttccgggaga

SEQ ID NO: 366 - DNA, 50 bp, synthetic construct
  source 1..50: mol_type = other DNA
gccaacgagtaggcgatagcgcgtggctttttctcccggttcgccgcgag

SEQ ID NO: 367 - DNA, 70 bp, synthetic construct
  source 1..70: mol_type = other DNA
acgggccacatcaactcattgatagacaatgcgtccactgcccgtttttctcgcggccatagccgtgggc

SEQ ID NO: 368 - DNA, 66 bp, synthetic construct
  source 1..66: mol_type = other DNA
gggccacatcaactcattgatagacaatgcgtccactgcccttttctcgcggccatagccgtgggc

SEQ ID NO: 369 - DNA, 58 bp, synthetic construct
  source 1..58: mol_type = other DNA
tacaggttctggggggtgggtggggaacctgttttttctcgcggccatagccgtgggc

SEQ ID NO: 370 - DNA, 61 bp, synthetic construct
  source 1..61: mol_type = other DNA
gccaacgagtaggcgatagcgcgtggctttttgctcctctcccggttcgccgcgagccgcg

SEQ ID NO: 371 - DNA, 74 bp, synthetic construct
  source 1..74: mol_type = other DNA
ctacgagacgaacttatgcgtaataatgactgtcgtagtttttcgcggctcgcggccatagccgtgggcgtcgc

SEQ ID NO: 372 - DNA, 64 bp, synthetic construct
  source 1..64: mol_type = other DNA
agccgcgagccgcgtttttacgggccacatcaactcattgatagacaatgcgtccactgcccgt

SEQ ID NO: 373 - DNA, 57 bp, synthetic construct
  source 1..57: mol_type = other DNA
agccgcgagccgcgtttttctacgagacgaacttatgcgtaataatgactgtcgtag

SEQ ID NO: 374 - DNA, 71 bp, synthetic construct
  source 1..71: mol_type = other DNA
ccactgcgggggtctatacgtgaggaagaagtggtttttgcgacgcccacgagcgttccgggagaggagct

SEQ ID NO: 375 - DNA, 61 bp, synthetic construct
  source 1..61: mol_type = other DNA
tcgtcgttttgtcgttttgtcgtttttttcgcggcacgcggccatagccgtgggcgtcgct

SEQ ID NO: 376 - DNA, 55 bp, synthetic construct
  source 1..55: mol_type = other DNA
tcgtcgttttgtcgttttgtcgtttttttgacgcccacgagcgttccgggagagg

SEQ ID NO: 377 - DNA, 67 bp, synthetic construct
  source 1..67: mol_type = other DNA
ccaacgagtaggcgatagcgcgtggtttttcctctcccggttcgccgcgagcctgtagcacggtggc

SEQ ID NO: 378 - DNA, 64 bp, synthetic construct
  source 1..64: mol_type = other DNA
acgggccacatcaactcattgatagacaatgcgtccactgcccgttttttgccaccgtgctaca

SEQ ID NO: 379 - DNA, 68 bp, synthetic construct
  source 1..68: mol_type = other DNA
tcgtcgttttgtcgttttgtcgttttttggctcgcggccatagccgtgggcgtctgctgctgctgctg

SEQ ID NO: 380 - DNA, 54 bp, synthetic construct
  source 1..54: mol_type = other DNA
gtggattgttgtgttctgttggtttttgtgttgtctttttcagcagcagcagca

SEQ ID NO: 381 - DNA, 61 bp, synthetic construct
  misc_feature 41..61: note = CD47 siRNA antisense strand
  source 1..61: mol_type = other DNA
  misc_feature 1..40: note = DNA
gtggattgttgtgttctgttggtttttgtgttgtctttttatatctctgggtaatcacctt

SEQ ID NO: 382 - DNA, 50 bp, synthetic construct
  misc_feature 1..21: note = CD47 siRNA sense strand
  source 1..50: mol_type = other DNA
  misc_feature 22..50: note = DNA
ggtgattacccagagatatttgctcctctcccggttcgccgcgagccgcg

SEQ ID NO: 383 - DNA, 59 bp, synthetic construct
  misc_feature 39..59: note = PD-L1 siRNA antisense strand
  source 1..59: mol_type = other DNA
  misc_feature 1..38: note = DNA
gccccagttatgctttccccctctgtctctttgtttttttgattctcagtgtgctggtt

SEQ ID NO: 384 - DNA, 52 bp, synthetic construct
  misc_feature 1..21: note = PD-L1 siRNA sense strand
  source 1..52: mol_type = other DNA
  misc_feature 22..52: note = DNA
ccagcacactgagaatcaattcgcggctcgcggccatagccgtgggcgtcgc

SEQ ID NO: 385 - DNA, 61 bp, synthetic construct
  source 1..61: mol_type = other DNA
tcgtcgttttgtcgttttgtcgtttttttcgcggctcgcggccatagccgtgggcgtcgct

SEQ ID NO: 386 - DNA, 96 bp, synthetic construct
  source 1..96: mol_type = other DNA
tcgtcgttttgtcgttttgtcgtttttttcgcggctcgcggccatagccgtgggcgtcgctttttccgctcgagctagtctgacaaagagaaacac

SEQ ID NO: 387 - DNA, 91 bp, synthetic construct
  source 1..91: mol_type = other DNA
tcgtcgttttgtcgttttgtcgtttttttgcgacgcccacgagcgttccgggagaggagcttttttggtgggggtggacgggccgggtaga

SEQ ID NO: 388 - DNA, 109 bp, synthetic construct
  source 1..109: mol_type = other DNA
ccaacgagtaggcgatagcgcgtggtttttgctcctctcccggttcgccgcgagccgcgtttttacgggccacatcaactcattgatagacaatgcgtccactgcccgt

SEQ ID NO: 389 - DNA, 99 bp, synthetic construct
  source 1..99: mol_type = other DNA
tcgtcgttttgtcgttttgtcgtttttttcgcggctcgcggccatagccgtgggcgtcgctttttccactgcgggggtctatacgtgaggaagaagtgg

SEQ ID NO: 390 - DNA, 34 bp, synthetic construct
  source 1..34: mol_type = other DNA
gataagctgcggcgcccacgagcgttccgggagc

SEQ ID NO: 391 - DNA, 62 bp, synthetic construct
  source 1..62: mol_type = other DNA
ctgcacttggcttggatttcagaagggagaccctttttgctcccggttcgccgccagccgcc

SEQ ID NO: 392 - DNA, 39 bp, synthetic construct
  source 1..39: mol_type = other DNA
gataagctggcggcaggcggccatagccgtgggcgccgc

SEQ ID NO: 393 - DNA, 38 bp, synthetic construct
  source 1..38: mol_type = other DNA
gataagctgcgacgcccacgagcgttccgggagaggag

SEQ ID NO: 394 - DNA, 59 bp, synthetic construct
  source 1..59: mol_type = other DNA
ggtggtggtggttgtggtggtggtggtttttctcctctcccggttcgccgcgagccgcg

SEQ ID NO: 395 - DNA, 39 bp, synthetic construct
  source 1..39: mol_type = other DNA
gataagctcgcggcacgcggccatagccgtgggcgtcgc

SEQ ID NO: 396 - DNA, 38 bp, synthetic construct
  source 1..38: mol_type = other DNA
gataagctgcggcgcccacgagcgttccgggagaggag

SEQ ID NO: 397 - DNA, 59 bp, synthetic construct
  source 1..59: mol_type = other DNA
ggtggtggtggttgtggtggtggtggtttttctcctctcccggttcgccgccagccgcc

SEQ ID NO: 398 - DNA, 55 bp, synthetic construct
  source 1..55: mol_type = other DNA
ggtggtggtggttgtggtggtggtggtttttgctcccggttcgccgccagccgcc

SEQ ID NO: 399 - DNA, 54 bp, synthetic construct
  source 1..54: mol_type = other DNA
ccaacgagtaggcgatagcgcgtggtttttgctcccggttcgccgccagccgcc

SEQ ID NO: 400 - DNA, 54 bp, synthetic construct
  source 1..54: mol_type = other DNA
gcagttgatcctttggataccctggtttttgctcccggttcgccgccagccgcc

SEQ ID NO: 401 - DNA, 51 bp, synthetic construct
  source 1..51: mol_type = other DNA
ccctcctacatagggtttttggcggcaggcggccatagccgtgggcgccgc

SEQ ID NO: 402 - DNA, 44 bp, synthetic construct
  source 1..44: mol_type = other DNA
ccctcctacatagggtttttgctcccggttcgccgccagccgcc

SEQ ID NO: 403 - DNA, 53 bp, synthetic construct
  misc_feature 32..53: note = 34 is U and 33 to 53 is survivin siRNA sense strand
  source 1..53: mol_type = other DNA
  misc_feature 1..31: note = DNA
ggcggcaggcggccatagccgtgggcgccgctgcaggttccttatctgtcatt

SEQ ID NO: 404 - DNA, 48 bp, synthetic construct
  source 1..48: mol_type = other DNA
ccctcctacatagggtttttctcctctcccggttcgccgccagccgcc

SEQ ID NO: 405 - DNA, 51 bp, synthetic construct
  misc_feature 39..51: note = survivin siRNA antisense strand
  source 1..51: mol_type = other DNA
  misc_feature 1..38: note = DNA
ggtggtggtggttgtggtggtggtggtttgtgacagataaggaacctgcag

SEQ ID NO: 406 - RNA, 75 nt, synthetic construct
  source 1..75: mol_type = other RNA
gcggcgcccacgagcgttccgggagaggccaagggaccgaaaaagacctgacttctatactaagtctacgttccc

SEQ ID NO: 407 - RNA, 54 nt, synthetic construct
  source 1..54: mol_type = other RNA
ggcctctcccggttcgccgccagccgccaagataagctgataagctgataagct

SEQ ID NO: 408 - RNA, 58 nt, synthetic construct
  source 1..58: mol_type = other RNA
ggcggctggcggccatagccgtgggcgccgcaaaagcaggttccttatctgtcacatt

SEQ ID NO: 409 - DNA, 55 bp, synthetic construct
  source 1..55: mol_type = other DNA
gataagctgataagctgataagctgcggcgcccacgagcgttccgggagaggcct

SEQ ID NO: 410 - DNA, 59 bp, synthetic construct
  source 1..59: mol_type = other DNA
acctggggagtattggggaggaaggtttttggcctctcccggttcgccgccagccgcct

SEQ ID NO: 411 - DNA, 69 bp, synthetic construct
  misc_feature 1..37: note = FGF2 RNA aptamer
  source 1..69: mol_type = other DNA
  misc_feature 38..69: note = DNA
gggatactagggcattaatgttaccagtgtagtccctggcggctggcggccatagccgtgggcgccgct

SEQ ID NO: 412 - DNA, 51 bp, synthetic construct
  misc_feature 39..51: note = survivin siRNA antisense strand
  source 1..51: mol_type = other DNA
  misc_feature 1..38: note = DNA
ggtggtggtggttgtggtggtggtggaatgtgacagataaggaacctgcag

SEQ ID NO: 413 - DNA, 75 bp, synthetic construct
  misc_feature 43..75: note = PSMA RNA aptamer
  source 1..75: mol_type = other DNA
  misc_feature 1..42: note = DNA
gcggcgcccacgagcgttccgggagaggccaagggaccgaaaaagacctgacttctatactaagtctacgttccc

SEQ ID NO: 414 - DNA, 60 bp, synthetic construct
  source 1..60: mol_type = other DNA
gataagctgataagctgataagcttttttgcggcgcccacgagcgttccgggagaggcct

SEQ ID NO: 415 - DNA, 60 bp, synthetic construct
  source 1..60: mol_type = other DNA
ggtggtggtggttgtggtggtggtggtttttggcctctcccggttcgccgccagccgcct

SEQ ID NO: 416 - DNA, 68 bp, synthetic construct
  source 1..68: mol_type = other DNA
ccgctcgagctagtctgacaaagagaaacactttttggcggctggcggccatagccgtgggcgccgct

SEQ ID NO: 417 - DNA, 51 bp, synthetic construct
  misc_feature 33..51: note = EpCAM RNA aptamer
  source 1..51: mol_type = other DNA
  misc_feature 1..32: note = DNA
gcggcgcccacgagcgttccgggagaggccaagcgactggttacccggtcg

SEQ ID NO: 418 - DNA, 54 bp, synthetic construct
  source 1..54: mol_type = other DNA
ggcctctcccggttcgccgccagccgccaagataagctgataagctgataagct

SEQ ID NO: 419 - DNA, 58 bp, synthetic construct
  misc_feature 36..58: note = survivin siRNA sense strand
  source 1..58: mol_type = other DNA
  misc_feature 1..35: note = DNA
ggcggctggcggccatagccgtgggcgccgcaaaagcaggttccttatctgtcacatt

SEQ ID NO: 420 - DNA, 79 bp, synthetic construct
  misc_feature 1..40: note = IL-4Ra RNA aptamer
  source 1..79: mol_type = other DNA
  misc_feature 41..79: note = DNA
aaaaagcaacagggtgctccatgcgcatggaacctgcgcggataagctgcggcgcccacgagcgttccgggagaggcct

SEQ ID NO: 421 - DNA, 94 bp, synthetic construct
  source 1..94: mol_type = other DNA
acattgctgcgtgatcgcctcacatgggtttgtctggtcgatttggaggtggtgggtggctttttggcctctcccggttcgccgccagccgcct

SEQ ID NO: 422 - DNA, 85 bp, synthetic construct
  source 1..85: mol_type = other DNA
acgggccacatcaactcattgatagacaatgcgtccactgcccgtgataagctggcggctggcggccatagccgtgggcgccgct

SEQ ID NO: 423 - DNA, 55 bp, synthetic construct
  misc_feature 35..55: note = ATAD2siRNA antisense strand
  source 1..55: mol_type = other DNA
  misc_feature 1..34: note = DNA
ggtggtggtggttgtggtggtggtgggataagctgcgtcgaagttgtaggatttt

SEQ ID NO: 424 - DNA, 38 bp, synthetic construct
  source 1..38: mol_type = other DNA
gcggcgcccacgagcgttccgggagaggccgataagct

SEQ ID NO: 425 - DNA, 74 bp, synthetic construct
  source 1..74: mol_type = other DNA
taacgctgaccttagctgcatggctttacatgttccagataagctggcctctcccggttcgccgccagccgcct

SEQ ID NO: 426 - DNA, 68 bp, synthetic construct
  misc_feature 58..68: note = ATAD2siRNA sense strand
  source 1..68: mol_type = other DNA
  misc_feature 1..57: note = DNA
gataagctggcggctggcggccatagccgtgggcgccgcgataagctaatcctacaacttcgacgctt

SEQ ID NO: 427 - DNA, 73 bp, synthetic construct
  source 1..73: mol_type = other DNA
tggtgggggtggacgggccgggtagagataagctgataagctgcggcgcccacgagcgttccgggagaggcct

SEQ ID NO: 428 - DNA, 85 bp, synthetic construct
  source 1..85: mol_type = other DNA
cggggaaagtcacggggggtttcagatgttctgatcggtgtggaggataagctggcggctggcggccatagccgtgggcgccgct

SEQ ID NO: 429 - DNA, 86 bp, synthetic construct
  source 1..86: mol_type = other DNA
ggtggtggtggttgtggtggtggtggtttttgataagctgataagctgataagctgcggcgcccacgagcgttccgggagaggcct

SEQ ID NO: 430 - DNA, 74 bp, synthetic construct
  misc_feature 1..40: note = IL-4Ra RNA aptamer
  source 1..74: mol_type = other DNA
  misc_feature 41..74: note = DNA
aaaaagcaacagggtgctccatgcgcatggaacctgcgcgtttttggcctctcccggttcgccgccagccgcct

SEQ ID NO: 431 - DNA, 96 bp, synthetic construct
  source 1..96: mol_type = other DNA
ggacacggcaaaggggtatagcctaccggaccgtgaacatggaatggtgtgctgcgtggtttttggcggctggcggccatagccgtgggcgccgct

SEQ ID NO: 432 - DNA, 59 bp, synthetic construct
  source 1..59: mol_type = other DNA
aacggagtgtggctaactcgagataagctgcggcgcccacgagcgttccgggagaggcc

SEQ ID NO: 433 - DNA, 59 bp, synthetic construct
  source 1..59: mol_type = other DNA
ggtggtggtggttgtggtggtggtggtttttggcctctcccggttcgccgccagccgcc

SEQ ID NO: 434 - DNA, 58 bp, synthetic construct
  misc_feature 1..19: note = EpCAM RNA aptamer
  source 1..58: mol_type = other DNA
  misc_feature 20..58: note = DNA
gcgactggttacccggtcggataagctggcggctggcggccatagccgtgggcgccgc

SEQ ID NO: 435 - DNA, 46 bp, synthetic construct
  source 1..46: mol_type = other DNA
gataagctgcgacgcccacgagcgttccgggagaggaggataagct

SEQ ID NO: 436 - DNA, 67 bp, synthetic construct
  source 1..67: mol_type = other DNA
ggtggtggtggttgtggtggtggtggtttttctcctctcccggttcgccgcgagccgcggataagct

SEQ ID NO: 437 - DNA, 61 bp, synthetic construct
  source 1..61: mol_type = other DNA
ccaacgagtaggcgatagcgcgtggtttttcgcggcacgcggccatagccgtgggcgtcgc

SEQ ID NO: 438 - DNA, 80 bp, synthetic construct
  misc_feature 1..40: note = IL-4Ra RNA aptamer
  source 1..80: mol_type = other DNA
  misc_feature 41..80: note = DNA
aaaaagcaacagggtgctccatgcgcatggaacctgcgcggataagctgcgacgcccacgagcgttccgggagaggagct

SEQ ID NO: 439 - DNA, 77 bp, synthetic construct
  source 1..77: mol_type = other DNA
agggaatcttgcctagggagggagtagcgaaagggctcagataagctgctcctctcccggttcgccgcgagccgcgt

SEQ ID NO: 440 - DNA, 85 bp, synthetic construct
  source 1..85: mol_type = other DNA
acgggccacatcaactcattgatagacaatgcgtccactgcccgtgataagctcgcggctcgcggccatagccgtgggcgtcgct

SEQ ID NO: 441 - DNA, 51 bp, synthetic construct
  misc_feature 31..51: note = TAPsiRNA antisense strand
  source 1..51: mol_type = other DNA
  misc_feature 1..30: note = DNA
ggtggtggtggttgtggtggtggtggaaaaattctgaaccgtgtgcagctt

SEQ ID NO: 442 - DNA, 61 bp, synthetic construct
  source 1..61: mol_type = other DNA
gcgacgcccacgagcgttccgggagaggagcaaaaggtggtggtggttgtggtggtggtgg

SEQ ID NO: 443 - DNA, 55 bp, synthetic construct
  source 1..55: mol_type = other DNA
gctcctctcccggttcgccgcgagccgcgaagataagctgataagctgataagct

SEQ ID NO: 444 - DNA, 54 bp, synthetic construct
  misc_feature 36..54: note = TAPsiRNA sense strand
  source 1..54: mol_type = other DNA
  misc_feature 1..35: note = DNA
cgcggctcgcggccatagccgtgggcgtcgcaaaagctgcacacggttcagaat

SEQ ID NO: 445 - DNA, 95 bp, synthetic construct
  source 1..95: mol_type = other DNA
agcggtgacggcacagacggtacagttcccgtccctgcactacacgtatgccgctgataagctgcgacgcccacgagcgttccgggagaggagct

SEQ ID NO: 446 - DNA, 64 bp, synthetic construct
  source 1..64: mol_type = other DNA
ggtggtggtggttgtggtggtggtgggataagctgctcctctcccggttcgccgcgagccgcgt

SEQ ID NO: 447 - DNA, 49 bp, synthetic construct
  source 1..49: mol_type = other DNA
tccatgacgttcctgacgtttttgcggcgcccacgagcgttccgggagc

SEQ ID NO: 448 - DNA, 63 bp, synthetic construct
  source 1..63: mol_type = other DNA
gggaggacgatgcggaggaagggtaggtttttgcgacgcccacgagcgttccgggagaggagc

SEQ ID NO: 449 - DNA, 66 bp, synthetic construct
  misc_feature 1..37: note = FGF2 RNA aptamer
  source 1..66: mol_type = other DNA
  misc_feature 38..66: note = DNA
gggatactagggcattaatgttaccagtgtagtccctgctcctctcccggttcgccgcgagccgcg

SEQ ID NO: 450 - DNA, 61 bp, synthetic construct
  source 1..61: mol_type = other DNA
catcaccaccagagccaacgtcgataagctcgcggctcgcggccatagccgtgggcgtcgc

SEQ ID NO: 451 - DNA, 80 bp, synthetic construct
  source 1..80: mol_type = other DNA
cggggaaagtcacggggggtttcagatgttctgatcggtgtggagtttttgctcctctcccggttcgccgcgagccgcgt

SEQ ID NO: 452 - RNA, 45 nt, synthetic construct
  source 1..45: mol_type = other RNA
ggtggaagagggatgggccgacgtgccgcatcagcagcagcagca

SEQ ID NO: 453 - DNA, 89 bp, synthetic construct
  source 1..89: mol_type = other DNA
agcggtgacggcacagacggtacagttcccgtccctgcactacacgtatgccgctaaagcgacgcccacgagcgttccgggagaggagc

SEQ ID NO: 454 - DNA, 72 bp, synthetic construct
  misc_feature 1..40: note = IL-4Ra RNA aptamer
  source 1..72: mol_type = other DNA
  misc_feature 41..72: note = DNA
aaaaagcaacagggtgctccatgcgcatggaacctgcgcgaaagctcctctcccggttcgccgcgagccgcg

SEQ ID NO: 455 - DNA, 74 bp, synthetic construct
  misc_feature 1..40: note = OX40 RNA aptamer
  source 1..74: mol_type = other DNA
  misc_feature 41..74: note = DNA
cagtctgcatcgtaggaatcgccaccgtatactttcccacaaacgcggctcgcggccatagccgtgggcgtcgc

SEQ ID NO: 456 - DNA, 89 bp, synthetic construct
  misc_feature 1..54: note = OX40 RNA aptamer
  source 1..89: mol_type = other DNA
  misc_feature 55..89: note = DNA
gggatgcggaaaaaagaacacttccgattagggcccaccctaacggccgcagactttttgctcctctcccggttcgccgcgagccgcgt

SEQ ID NO: 457 - DNA, 82 bp, synthetic construct
  source 1..82: mol_type = other DNA
acgggccacatcaactcattgatagacaatgcgtccactgcccgttttttcgcggctcgcggccatagccgtgggcgtcgct

SEQ ID NO: 458 - DNA, 62 bp, synthetic construct
  misc_feature 1..27: note = VEGF165 RNA aptamer
  source 1..62: mol_type = other DNA
  misc_feature 28..62: note = DNA
cggaatcagtgaatgcttatacatccgtttttgctcctctcccggttcgccgcgagccgcgt

SEQ ID NO: 459 - DNA, 98 bp, synthetic construct
  misc_feature 1..61: note = TIM3 RNA aptamer
  source 1..98: mol_type = other DNA
  misc_feature 62..98: note = DNA
gggagaggaccagtagccactatggtgttggagctagcggcagagcgtcgcggtccctccctttttcgcggctcgcggccatagccgtgggcgtcgct

SEQ ID NO: 460 - DNA, 92 bp, synthetic construct
  source 1..92: mol_type = other DNA
agcggtgacggcacagacggtacagttcccgtccctgcactacacgtatgccgcttttttgcgacgcccacgagcgttccgggagaggagct

SEQ ID NO: 461 - DNA, 107 bp, synthetic construct
  misc_feature 1..70: note = LAG3 RNA aptamer
  source 1..107: mol_type = other DNA
  misc_feature 71..107: note = DNA
gggagagagatataagggcctcctgatacccgctgctatctggaccgatcccattaccaaattctctccctttttcgcggctcgcggccatagccgtgggcgtcgct

SEQ ID NO: 462 - DNA, 62 bp, synthetic construct
  source 1..62: mol_type = other DNA
gaagtgaaaatgacagaacacaacatttttcgcggctcgcggccatagccgtgggcgtcgct

SEQ ID NO: 463 - DNA, 95 bp, synthetic construct
  source 1..95: mol_type = other DNA
acattgctgcgtgatcgcctcacatgggtttgtctggtcgatttggaggtggtgggtggctttttgctcctctcccggttcgccgcgagccgcgt

SEQ ID NO: 464 - DNA, 60 bp, synthetic construct
  source 1..60: mol_type = other DNA
ccaacgagtaggcgatagcgcgtggtttttgctcctctcccggttcgccgcgagccgcgt

SEQ ID NO: 465 - DNA, 68 bp, synthetic construct
  misc_feature 1..30: note = CTLA-4 RNA aptamer
  source 1..68: mol_type = other DNA
  misc_feature 31..68: note = DNA
ggtggaagagggatgggccgacgtgccgcattttttcgcggctcgcggccatagccgtgggcgtcgct

SEQ ID NO: 466 - DNA, 83 bp, synthetic construct
  misc_feature 1..49: note = HER3 RNA aptamer
  source 1..83: mol_type = other DNA
  misc_feature 50..83: note = DNA
cagcgaaagttgcgtatgggtcacatcgcaggcacatgtcatctgggcgaagcgacgcccacgagcgttccgggagaggagct

SEQ ID NO: 467 - DNA, 92 bp, synthetic construct
  source 1..92: mol_type = other DNA
ccaacgagtaggcgatagcgcgtggaagctcctctcccggttcgccgcgagccgcgaaccactgcgggggtctatacgtgaggaagaagtgg

SEQ ID NO: 468 - DNA, 68 bp, synthetic construct
  source 1..68: mol_type = other DNA
  misc_feature 1..34: note = HER2 RNA aptamer
  misc_feature 35..68: note = DNA
agccgcgaggggagggatagggtagggcgcggctaacgcggctcgcggccatagccgtgggcgtcgct

SEQ ID NO: 469 - DNA, 89 bp, synthetic construct
  misc_feature 1..31: note = CTLA-4 RNA aptamer
  source 1..89: mol_type = other DNA
  misc_feature 32..89: note = DNA
ggtggaagagggatgggccgacgtgccgcattttcgcggctcgcggccatagccgtgggcgtcgctttaacggagtgtggctaactcga

SEQ ID NO: 470 - DNA, 84 bp, synthetic construct
  misc_feature 1..59: note = HER3 RNA aptamer
  source 1..84: mol_type = other DNA
  misc_feature 60..84: note = DNA
cagcgaaagttgcgtatgggtcacatcgcaggcacatgtcatctgggcgtttttgctcctctcccggttcgccgcgagccgcgt

SEQ ID NO: 471 - DNA, 64 bp, synthetic construct
  misc_feature 1..27: note = VEGF165 RNA aptamer
  source 1..64: mol_type = other DNA
  misc_feature 28..64: note = DNA
cggaatcagtgaatgcttatacatccgtttttcgcggctcgcggccatagccgtgggcgtcgct

SEQ ID NO: 472 - DNA, 89 bp, synthetic construct
  source 1..89: mol_type = other DNA
ggtgggggtggacgggccgggtagattttttgcgacgcccacgagcgttccgggagaggagcttttttaacggagtgtggctaactcga

SEQ ID NO: 473 - DNA, 80 bp, synthetic construct
  source 1..80: mol_type = other DNA
acgggccacatcaactcattgatagacaatgcgtccactgcccgttttttgctcctctcccggttcgccgcgagccgcgt

SEQ ID NO: 474 - DNA, 71 bp, synthetic construct
  source 1..71: mol_type = other DNA
ccactgcgggggtctatacgtgaggaagaagtggtttttcgcggctcgcggccatagccgtgggcgtcgct

SEQ ID NO: 475 - DNA, 83 bp, synthetic construct
  source 1..83: mol_type = other DNA
acgggccacatcaactcattgatagacaatgcgtccactgcccgtgataagctgctcctctcccggttcgccgcgagccgcgt

SEQ ID NO: 476 - DNA, 82 bp, synthetic construct
  source 1..82: mol_type = other DNA
cggggaaagtcacggggggtttcagatgttctgatcggtgtggagtttttcgcggctcgcggccatagccgtgggcgtcgct

SEQ ID NO: 477 - DNA, 74 bp, synthetic construct
  source 1..74: mol_type = other DNA
cagcgaaagttgcgtatgggtcacatcgcaggcacatgtcatctgggcgaaaattagataagactgctaaggca

SEQ ID NO: 478 - DNA, 60 bp, synthetic construct
  source 1..60: mol_type = other DNA
gcggcgcccacgagcgttccgggagaggccaaaaggtggtggtggttgtggtggtggtgg

SEQ ID NO: 479 - DNA, 53 bp, synthetic construct
  misc_feature 33..53: note = EGFR siRNA sense strand
  source 1..53: mol_type = other DNA
  misc_feature 1..32: note = DNA
ggcctctcccggttcgccgccagccgccaaaagcaggttccttatctgtcaca

SEQ ID NO: 480 - RNA, 59 nt, synthetic construct
  source 1..59: mol_type = other RNA
agccgcgaggggagggatagggtagggcgcggctaatgtgacagataaggaacctgcag

SEQ ID NO: 481 - DNA, 56 bp, synthetic construct
  misc_feature 36..56: note = EGFR siRNA sense strand
  source 1..56: mol_type = other DNA
  misc_feature 1..35: note = DNA
ggcggctggcggccatagccgtgggcgccgcaaaaccttagcagtcttatctaatt

SEQ ID NO: 482 - DNA, 52 bp, synthetic construct
  source 1..52: mol_type = other DNA
gcgtggtcacacgcggataagctcgacgcccacgagcgttccgggagaggag

SEQ ID NO: 483 - DNA, 62 bp, synthetic construct
  source 1..62: mol_type = other DNA
ggtggtggtggttgtggtggtggtgggataagctctcctctcccggttcgccgccagccgcc

SEQ ID NO: 484 - DNA, 58 bp, synthetic construct
  misc_feature 1..19: note = Survivin siRNA sense strand
  source 1..58: mol_type = other DNA
  misc_feature 20..58: note = DNA
gcaggttccttatctgtcagataagctggcggcaggcggccatagccgtgggcgccgc

SEQ ID NO: 485 - DNA, 51 bp, synthetic construct
  source 1..51: mol_type = other DNA
  misc_feature 29..51: note = EGFR siRNA antisense strand
  misc_feature 1..28: note = DNA
ggtggtggtggttgtggtggtggtggaaaattagataagactgctaaggca

SEQ ID NO: 486 - RNA, 59 nt, synthetic construct
  source 1..59: mol_type = other RNA
gcggcgcccacgagcgttccgggagaggccaacggaatcagtgaatgcttatacatccg

SEQ ID NO: 487 - DNA, 75 bp, synthetic construct
  misc_feature 1..28: note = RNA type b sequence
  source 1..75: mol_type = other DNA
  misc_feature 29..75: note = DNA
ggcctctcccggttcgccgccagccgccaaacgggccacatcaactcattgatagacaatgcgtccactgcccgt

SEQ ID NO: 488 - RNA, 54 nt, synthetic construct
  source 1..54: mol_type = other RNA
ggcggctggcggccatagccgtgggcgccgcaaccttagcagtcttatctaatt

SEQ ID NO: 489 - DNA, 86 bp, synthetic construct
  source 1..86: mol_type = other DNA
ttaacttattcgaccataaagcggcgcccacgagcgttccgggagaggccaaccactgcgggggtctatacgtgaggaagaagtgg

SEQ ID NO: 490 - DNA, 76 bp, synthetic construct
  source 1..76: mol_type = other DNA
cggggaaagtcacggggggtttcagatgttctgatcggtgtggagaaggcctctcccggttcgccgccagccgcct

SEQ ID NO: 491 - DNA, 79 bp, synthetic construct
  source 1..79: mol_type = other DNA
acgggccacatcaactcattgatagacaatgcgtccactgcccgtaaggcggctggcggccatagccgtgggcgccgct

SEQ ID NO: 492 - DNA, 50 bp, synthetic construct
  misc_feature 30..50: note = TAP siRNA antisense strand
  source 1..50: mol_type = other DNA
  misc_feature 1..29: note = DNA
ggtggtggtggttgtggtggtggtggaaaattctgaaccgtgtgcagctt

SEQ ID NO: 493 - DNA, 68 bp, synthetic construct
  source 1..68: mol_type = other DNA
gcggcgcccacgagcgttccgggagaggccaaaaccactgcgggggtctatacgtgaggaagaagtgg

SEQ ID NO: 494 - DNA, 63 bp, synthetic construct
  misc_feature 33..63: note = CTLA-4 RNA aptamer
  source 1..63: mol_type = other DNA
  misc_feature 1..32: note = DNA
ggcctctcccggttcgccgccagccgccaaaaggtggaagagggatgggccgacgtgccgcat

SEQ ID NO: 495 - DNA, 54 bp, synthetic construct
  misc_feature 34..54: note = TAP siRNA sense strand
  source 1..54: mol_type = other DNA
  misc_feature 1..33: note = DNA
ggcggctggcggccatagccgtgggcgccgcaaaagctgcacacggttcagaat

SEQ ID NO: 496 - DNA, 86 bp, synthetic construct
  source 1..86: mol_type = other DNA
ggcctctcccggttcgccgccagccgccaaaacggggaaaacggggaaagtcacggggggtttcagatgttctgatcggtgtggag

SEQ ID NO: 497 - DNA, 87 bp, synthetic construct
  misc_feature 69..87: note = TAP siRNA sense strand
  source 1..87: mol_type = other DNA
  misc_feature 1..68: note = DNA
ccactgcgggggtctatacgtgaggaagaagtggaagcggcgcccacgagcgttccgggagaggccaagctgcacacggttcagaat

SEQ ID NO: 498 - DNA, 99 bp, synthetic construct
  misc_feature 31..99: note = OX40 RNA aptamer
  source 1..99: mol_type = other DNA
  misc_feature 1..30: note = DNA
ggcctctcccggttcgccgccagccgccaagggaggacgatgcggcagtctgcatcgtaggaatcgccaccgtatactttcccaccagacgactcgctg

SEQ ID NO: 499 - DNA, 80 bp, synthetic construct
  source 1..80: mol_type = other DNA
cggggaaagtcacggggggtttcagatgttctgatcggtgtggagaaaaggcggctggcggccatagccgtgggcgccgc

SEQ ID NO: 500 - DNA, 67 bp, synthetic construct
  misc_feature 1..31: note = CTLA-4 RNA aptamer
  source 1..67: mol_type = other DNA
  misc_feature 32..67: note = DNA
ggtggaagagggatgggccgacgtgccgcattttttgcggcgcccacgagcgttccgggagaggcct

SEQ ID NO: 501 - DNA, 59 bp, synthetic construct
  source 1..59: mol_type = other DNA
ccaacgagtaggcgatagcgcgtggtttttggcctctcccggttcgccgccagccgcct

SEQ ID NO: 502 - DNA, 50 bp, synthetic construct
  source 1..50: mol_type = other DNA
cggaatcagtgaatgcttatacatccgaatgatattatggaagcaaattt

SEQ ID NO: 503 - DNA, 90 bp, synthetic construct
  source 1..90: mol_type = other DNA
gcggcgcccacgagcgttccgggagaggccaagctggatgtcgcttacgacaatattccttaggggcaccgctacattgacacatccagc

SEQ ID NO: 504 - DNA, 106 bp, synthetic construct
  source 1..106: mol_type = other DNA
ggcctctcccggttcgccgccagccgccaaatccagagtgacgcagcatatgtgggtgggtgggcggttatgctgagtcagccttgcttggacacggtggcttagt

SEQ ID NO: 505 - DNA, 54 bp, synthetic construct
  misc_feature 34..54: note = ASAP1siRNA sense strand
  source 1..54: mol_type = other DNA
  misc_feature 1..33: note = DNA
ggcggctggcggccatagccgtgggcgccgcaaatttgcttccataatatcatt

SEQ ID NO: 506 - DNA, 88 bp, synthetic construct
  misc_feature 1..56: note = FGF5 RNA aptamer
  source 1..88: mol_type = other DNA
  misc_feature 57..88: note = DNA
gggcgacctctccgtactgacctacagagcgacatactagtgtatccagatcgccctgcggcgcccacgagcgttccgggagaggcct

SEQ ID NO: 507 - DNA, 85 bp, synthetic construct
  misc_feature 1..56: note = FGF5 RNA aptamer
  source 1..85: mol_type = other DNA
  misc_feature 57..85: note = DNA
ggcgacctctccgtactgacctacagagcgacatactagtgtatccagatcgccctggcctctcccggttcgccgccagccgcct

SEQ ID NO: 508 - DNA, 89 bp, synthetic construct
  misc_feature 1..56: note = FGF5 RNA aptamer
  source 1..89: mol_type = other DNA
  misc_feature 57..89: note = DNA
gggcgacctctccgtactgacctacagagcgacatactagtgtatccagatcgccctggcggctggcggccatagccgtgggcgccgct

SEQ ID NO: 509 - DNA, 49 bp, synthetic construct
  misc_feature 29..49: note = ASAP1 siRNA antisense strand
  source 1..49: mol_type = other DNA
  misc_feature 1..28: note = DNA
ggtggtggtggttgtggtggtggtggaatgatattatggaagcaaattt

SEQ ID NO: 510 - DNA, 59 bp, synthetic construct
  misc_feature 33..59: note = VEGF165 RNA aptamer
  source 1..59: mol_type = other DNA
  misc_feature 1..32: note = DNA
gcggcgcccacgagcgttccgggagaggccaacggaatcagtgaatgcttatacatccg

SEQ ID NO: 511 - DNA, 88 bp, synthetic construct
  source 1..88: mol_type = other DNA
ggcctctcccggttcgccgccagccgccaagctggatgtcgcttacgacaatattccttaggggcaccgctacattgacacatccagc

SEQ ID NO: 512 - RNA, 54 nt, synthetic construct
  source 1..54: mol_type = other RNA
ggcggctggcggccatagccgtgggcgccgcaaatttgcttccataatatcatt

SEQ ID NO: 513 - DNA, 76 bp, synthetic construct
  source 1..76: mol_type = other DNA
accgacagtgaaggactcagcgaactctcagactcggttctttttcgcggctcgcggccatagccgtgggcgtcgc

SEQ ID NO: 514 - DNA, 77 bp, synthetic construct
  source 1..77: mol_type = other DNA
tatgtgggtgggtgggcggttatgctgagtcagccttgctgtcgttgcgacgcccacgagcgttccgggagaggagc

SEQ ID NO: 515 - DNA, 44 bp, synthetic construct
  misc_feature 23..44: note = 23 is U and 24 to 44 is HBVsiRNA sense strand
  source 1..44: mol_type = other DNA
  misc_feature 1..22: note = DNA
cgcccacgagcgttccgggagatggacttctctcaattttcttt

SEQ ID NO: 516 - DNA, 62 bp, synthetic construct
  misc_feature 41..62: note = 41 is U and 42 to 62 is HBVsiRNA antisense strand
  source 1..62: mol_type = other DNA
  misc_feature 1..40: note = DNA
cacagcgaacagcggcggacataatagtgcttactacgactagaaaattgagagaagtcctt

SEQ ID NO: 517 - DNA, 67 bp, synthetic construct
  source 1..67: mol_type = other DNA
tctcccggttcgccgcgagtgtgacagaacaacgtataacaatgcccacgtcaccagagtactatgg

SEQ ID NO: 518 - DNA, 57 bp, synthetic construct
  source 1..57: mol_type = other DNA
ctcgcggccatagccgtgggcgtggcagtgtggtggtggtggttgtggtggtggtgg

SEQ ID NO: 519 - RNA, 63 nt, synthetic construct
  source 1..63: mol_type = other RNA
aaaaagcaacagggtgctccatgcgcatggaacctgcgcgtcgcccacgagcgttccgggaga

SEQ ID NO: 520 - RNA, 57 nt, synthetic construct
  source 1..57: mol_type = other RNA
aagcaacacttagtcgcgattgatacgtgcgcagtcattctcccggttcgccgcgag

SEQ ID NO: 521 - RNA, 51 nt, synthetic construct
  source 1..51: mol_type = other RNA
tcgtacctcgtacctcgtacctcgtacctctcgcggccatagccgtgggcg

SEQ ID NO: 522 - DNA, 83 bp, synthetic construct
  misc_feature 1..52: note = 1 to 50 is BCMA RNA aptamer and 51 to 55 is UU
  source 1..83: mol_type = other DNA
  misc_feature 53..83: note = DNA
agtgcaagacgttcgcagattagcgaaaagagggtctcattgactagtacaagcgacgcccacgagcgttccgggagaggagc

SEQ ID NO: 523 - DNA, 39 bp, synthetic construct
  source 1..39: mol_type = other DNA
gataagctgcgacgcccacgagcgttccgggagaggagc

SEQ ID NO: 524 - DNA, 40 bp, synthetic construct
  source 1..40: mol_type = other DNA
gataagctcgcggctcgcggccatagccgtgggcgtcgct

SEQ ID NO: 525 - DNA, 63 bp, synthetic construct
  source 1..63: mol_type = other DNA
cctgcacttggcttggatttcagaagggagaccctttttgctcccggttcgccgccagccgcc

SEQ ID NO: 526 - DNA, 49 bp, synthetic construct
  misc_feature 27..49: note = Survivin siRNA sense strand
  source 1..49: mol_type = other DNA
  misc_feature 1..26: note = DNA
gcggcgcccacgagcgttccgggagcgcaggttccttatctgtcacatt

SEQ ID NO: 527 - DNA, 54 bp, synthetic construct
  misc_feature 32..54: note = Survivin siRNA sense strand
  source 1..54: mol_type = other DNA
  misc_feature 1..31: note = DNA
ggcggcaggcggccatagccgtgggcgccgcgcaggttccttatctgtcacatt

SEQ ID NO: 528 - DNA, 70 bp, synthetic construct
  source 1..70: mol_type = other DNA
ccactgcgggggtctatacgtgaggaagaagtggtttttgcgacgcccacgagcgttccgggagaggagc

SEQ ID NO: 529 - DNA, 60 bp, synthetic construct
  source 1..60: mol_type = other DNA
tcgtcgttttgtcgttttgtcgtttttttcgcggctcgcggccatagccgtgggcgtcgc

SEQ ID NO: 530 - DNA, 57 bp, synthetic construct
  source 1..57: mol_type = other DNA
tcgtcgttttgtcgttttgtcgtttttttgcgacgcccgcagcgttcgggagaggag

SEQ ID NO: 531 - DNA, 57 bp, synthetic construct
  source 1..57: mol_type = other DNA
ccaacgagtaggcgatagcgcgtggtttttctcctctcccgttcgccgcgagccgcg

SEQ ID NO: 532 - DNA, 59 bp, synthetic construct
  source 1..59: mol_type = other DNA
tcgtcgttttgtcgttttgtcgtttttttcgcggcacgcggccatagcgcgggcgtcgc

SEQ ID NO: 533 - DNA, 36 bp, synthetic construct
  source 1..36: mol_type = other DNA
gataagctgcgacgcccgcagcgttcgggagaggag

SEQ ID NO: 534 - DNA, 58 bp, synthetic construct
  source 1..58: mol_type = other DNA
ggtggtggtggttgtggtggtggtggtttttctcctctcccgttcggcccgagccgcg

SEQ ID NO: 535 - DNA, 38 bp, synthetic construct
  source 1..38: mol_type = other DNA
gataagctcgcggcacgggcccatagcgcgggcgtcgc